European Patent Specification EP 3 630 147 B1, published March 25, 2026. Title: PEPTIDE PAC1 ANTAGONISTS. Applicant: AMGEN INC. Harrington, Essa Hu. The sequence listing filed with the application follows.

SEQUENCE LISTING (451 sequences)

SEQ ID NO: 1 - protein, 43 aa, Artificial Sequence
  Synthetic Polypeptide
  DISULFID (1)..(5)
  DISULFID (14)..(31)
  MOD_RES (43)..(43): C-terminal amidation
CDATCQFRKAIDDCAKASWHSNVPGSVFKSCMKQKKKEWKAGH

SEQ ID NO: 2 - protein, 43 aa, Artificial Sequence
  Synthetic Polypeptide
  DISULFID (1)..(5)
  DISULFID (14)..(31)
  MOD_RES (43)..(43): C-terminal amidation
CDATCQFRKAIDDCARQAHHSNVPGSVFKACMKQKKKEWKAGH

SEQ ID NO: 3 - protein, 39 aa, Artificial Sequence
  Synthetic Polypeptide
  DISULFID (1)..(5)
  DISULFID (14)..(27)
CDATCQFRKAIDDCVRQAHHSSVFKACMKQKKKEWKAGY

SEQ ID NO: 4 - skipped

SEQ ID NO: 5 - protein, 35 aa, Artificial Sequence
  Synthetic Polypeptide
  DISULFID (1)..(5)
  DISULFID (14)..(27)
  MOD_RES (35)..(35): C-terminal amidation
CDATCQYRKGLVACARQAYHSSVFKACMKQKKKEW

SEQ ID NO: 6 - protein, 38 aa, Artificial Sequence
  Synthetic Polypeptide
  DISULFID (1)..(5)
  DISULFID (14)..(27)
  MOD_RES (28)..(28): Xaa = selenomethionine amino acid
  MOD_RES (38)..(38): C-terminal amidation
CDATCQFRKAIDDCARQAYHSSVFKACXKQKKKEWKAG

SEQ ID NO: 7 - protein, 43 aa, Artificial Sequence
  Synthetic Polypeptide
  DISULFID (1)..(5)
  DISULFID (14)..(31)
  MOD_RES (32)..(32): Xaa = selenomethionine amino acid
CDATCQFRKAIDDCARQAHHSNVPGSVFKACXKQKKKEWKAGH

SEQ ID NO: 8 - protein, 43 aa, Artificial Sequence
  Synthetic Polypeptide
  DISULFID (1)..(5)
  DISULFID (14)..(31)
CDATCQFRKAIDDCARQAHHANVPGSVFKACMKQKKKEWKAGH

SEQ ID NO: 9 - protein, 43 aa, Artificial Sequence
  Synthetic Polypeptide
  DISULFID (1)..(5)
  DISULFID (14)..(31)
CDATCQFRKAIDDCARQAHHSNVPGSVFKACIKQKKKEWKAGH

SEQ ID NO: 10 - protein, 43 aa, Artificial Sequence
  Synthetic Polypeptide
  DISULFID (1)..(5)
  DISULFID (14)..(31)
CDATCQFRKAIDDCARQAHHSNVPGSVFKACMKQKKKEYKAGH

SEQ ID NO: 11 - protein, 43 aa, Artificial Sequence
  Synthetic Polypeptide
  DISULFID (1)..(5)
  DISULFID (14)..(31)
CEATCQFRKAIDDCARQAHHSNVPGSVFKACMKQKKKEWKAGH

SEQ ID NO: 12 - protein, 42 aa, Artificial Sequence
  Synthetic Polypeptide
  DISULFID (1)..(5)
  DISULFID (14)..(31)
  MOD_RES (42)..(42): C-terminal amidation
CDATCQFRKAIDECAKQAHHSNVPGSVFKACMKQKKKEFKAG

SEQ ID NO: 13 - protein, 42 aa, Artificial Sequence
  Synthetic Polypeptide
  DISULFID (1)..(5)
  DISULFID (14)..(31)
  MOD_RES (42)..(42): C-terminal amidation
CDATCQFRKAIDDCAKQAHHANVPGSVFKACMKQKKKEFKAG

SEQ ID NO: 14 - protein, 42 aa, Artificial Sequence
  Synthetic Polypeptide
  DISULFID (1)..(5)
  DISULFID (14)..(31)
  MOD_RES (42)..(42): C-terminal amidation
CDATCQFRKAIDDCAKQAHHSNVPGSVFKACIKQKKKEFKAG

SEQ ID NO: 15 - protein, 40 aa, Artificial Sequence
  Synthetic Polypeptide
  DISULFID (2)..(6)
  DISULFID (15)..(28)
GCDATCQFRKAIDDCVRQAHHSSVFKACMKQKKKEWKAGH

SEQ ID NO: 16 - protein, 38 aa, Artificial Sequence
  Synthetic Polypeptide
  DISULFID (1)..(5)
  DISULFID (14)..(27)
  MOD_RES (38)..(38): C-terminal amidation
CDATCQFRKAIDDCDRQAHHSSVFKACMKQKKKEWKAG

SEQ ID NO: 17 - protein, 42 aa, Artificial Sequence
  Synthetic Polypeptide
  DISULFID (1)..(5)
  DISULFID (14)..(31)
  MOD_RES (42)..(42): C-terminal amidation
CDATCQFRKAIDDCARQAHHSNVPGSVFKACMKQKKKEFKAG

SEQ ID NO: 18 - protein, 42 aa, Artificial Sequence
  Synthetic Polypeptide
  DISULFID (1)..(5)
  DISULFID (14)..(31)
  MOD_RES (42)..(42): C-terminal amidation
CDATCQFRKAIDDCAKQAHHSNVPGSVFKLCMKQKKKEFKAG

SEQ ID NO: 19 - protein, 39 aa, Artificial Sequence
  Synthetic Polypeptide
  DISULFID (1)..(5)
  DISULFID (14)..(27)
CDATCQFRKAIDDCVKQAHHSSVFKACMKQKKKEFKAGH

SEQ ID NO: 20 - protein, 37 aa, Artificial Sequence
  Synthetic Polypeptide
  DISULFID (1)..(5)
  DISULFID (14)..(26)
  MOD_RES (37)..(37): C-terminal amidation
CDATCQFRKAIDDCARQAYHSSFKACMKQKKKEWKAG

SEQ ID NO: 21 - protein, 38 aa, Artificial Sequence
  Synthetic Polypeptide
  DISULFID (1)..(5)
  DISULFID (14)..(27)
  MOD_RES (21)..(21): C-terminal amidation
CDATCQFRKAIDDCDRQAYHSSVFKACMKQKKKEWKAG

SEQ ID NO: 22 - protein, 43 aa, Artificial Sequence
  Synthetic Polypeptide
  DISULFID (1)..(5)
  DISULFID (14)..(31)
CDATCQFRKAIDDCARQAHHSQVPGSVFKACMKQKKKEWKAGH

SEQ ID NO: 23 - protein, 43 aa, Artificial Sequence
  Synthetic Polypeptide
  DISULFID (1)..(5)
  DISULFID (14)..(31)
CDATCQFRKAIDDCARQAHHSNVPGSVFKLCMKQKKKEWKAGH

SEQ ID NO: 24 - protein, 43 aa, Artificial Sequence
  Synthetic Polypeptide
  DISULFID (1)..(5)
  DISULFID (14)..(31)
CDATCQFRKAIDDCARQAHHSNVPGSVFKSCMKQKKKEWKAGH

SEQ ID NO: 25 - protein, 43 aa, Artificial Sequence
  Synthetic Polypeptide
  DISULFID (1)..(5)
  DISULFID (14)..(31)
CDATCQFRKAIDECARQAHHSNVPGSVFKACMKQKKKEWKAGH

SEQ ID NO: 26 - protein, 39 aa, Artificial Sequence
  Synthetic Polypeptide
  DISULFID (1)..(5)
  DISULFID (14)..(27)
CDATCQFRKAIDDCAKQAHHSSVFKACMKQKKKEWKAGH

SEQ ID NO: 27 - protein, 39 aa, Artificial Sequence
  Synthetic Polypeptide
  DISULFID (1)..(5)
  DISULFID (14)..(27)
CDATCQFRKAIDDCARQAYHSSVFKACMKQKKKEWKAGH

SEQ ID NO: 28 - protein, 39 aa, Artificial Sequence
  Synthetic Polypeptide
  DISULFID (1)..(5)
  DISULFID (14)..(27)
CDATCQFRKAIDDCARQAHHSSVFKACMKQKKKEWKAGH

SEQ ID NO: 29 - protein, 39 aa, Artificial Sequence
  Synthetic Polypeptide
  DISULFID (1)..(5)
  DISULFID (14)..(27)
CDATCQFRKAIDDCAKQAHHSSVFKACMKQKKKEFKAGY

SEQ ID NO: 30 - protein, 39 aa, Artificial Sequence
  Synthetic Polypeptide
  DISULFID (1)..(5)
  DISULFID (14)..(27)
CDATCQFRKAIDDCAKQAYHSSVFKACMKQKKKEFKAGY

SEQ ID NO: 31 - protein, 42 aa, Artificial Sequence
  Synthetic Polypeptide
  DISULFID (1)..(5)
  DISULFID (14)..(31)
  MOD_RES (42)..(42): C-terminal amidation
CDATCQFRKAIDDCAKQAHHSNVPGSVFKSCMKQKKKEFKAG

SEQ ID NO: 32 - protein, 42 aa, Artificial Sequence
  Synthetic Polypeptide
  DISULFID (1)..(5)
  DISULFID (14)..(31)
  MOD_RES (18)..(18): Xaa = propargylglycine
  MOD_RES (42)..(42): C-terminal amidation
CDATCQFRKAIDDCQKQXHHSNVPGSVFKACMKQKKKEFKAG

SEQ ID NO: 33 - protein, 42 aa, Artificial Sequence
  Synthetic Polypeptide
  DISULFID (1)..(5)
  DISULFID (14)..(31)
  MOD_RES (16)..(16): Xaa = propargylglycine
  MOD_RES (42)..(42): C-terminal amidation
CDATCQFRKAIDDCQXQAHHSNVPGSVFKACMKQKKKEFKAG

SEQ ID NO: 34 - protein, 42 aa, Artificial Sequence
  Synthetic Polypeptide
  DISULFID (1)..(5)
  DISULFID (14)..(31)
  MOD_RES (26)..(26): Xaa = propargylglycine
  MOD_RES (42)..(42): C-terminal amidation
CDATCQFRKAIDDCQKQAHHSNVPXSVFKACMKQKKKEFKAG

SEQ ID NO: 35 - protein, 39 aa, Artificial Sequence
  Synthetic Polypeptide
  DISULFID (1)..(5)
  DISULFID (14)..(27)
CDATCQFRKAIDDCARQAYHSSVFKACMKQKKKEFKAGH

SEQ ID NO: 36 - protein, 39 aa, Artificial Sequence
  Synthetic Polypeptide
  DISULFID (1)..(5)
  DISULFID (14)..(27)
CDATCQFRKAIDDCARQAHHSSVFKACMKQKKKEFKAGH

SEQ ID NO: 37 - protein, 38 aa, Artificial Sequence
  Synthetic Polypeptide
  DISULFID (1)..(5)
  DISULFID (14)..(26)
CDATCQFRKAIDDCAKQAHSSVFKACMKQKKKEFKAGY

SEQ ID NO: 38 - skipped

SEQ ID NO: 39 - protein, 43 aa, Artificial Sequence
  Synthetic Polypeptide
  DISULFID (1)..(5)
  DISULFID (14)..(31)
CDATCQFRKAIDDCARQAHHSNVPGSVFKACFKQKKKEWKAGH

SEQ ID NO: 40 - protein, 43 aa, Artificial Sequence
  Synthetic Polypeptide
  DISULFID (1)..(5)
  DISULFID (14)..(31)
CDATCQFRKAIDDCARQAHHSNVPGSVFKACSKQKKKEWKAGH

SEQ ID NO: 41 - protein, 43 aa, Artificial Sequence
  Synthetic Polypeptide
  DISULFID (1)..(5)
  DISULFID (14)..(31)
CDATCQFRKAIDDCARQAHHSNVPGSVFKACLKQKKKEWKAGH

SEQ ID NO: 42 - protein, 41 aa, Artificial Sequence
  Synthetic Polypeptide
  DISULFID (1)..(5)
  DISULFID (14)..(30)
  MOD_RES (41)..(41): C-terminal amidation
CDATCQFRKAIDDCYYRSHSNVPGSVFKACMKQKKKEFKAG

SEQ ID NO: 43 - protein, 42 aa, Artificial Sequence
  Synthetic Polypeptide
  DISULFID (1)..(5)
  DISULFID (14)..(31)
  MOD_RES (42)..(42): C-terminal amidation
CDATCQFRKAIDDCYYRSKHSNVPGSVFKACMKQKKKEFKAG

SEQ ID NO: 44 - protein, 42 aa, Artificial Sequence
  Synthetic Polypeptide
  DISULFID (1)..(5)
  DISULFID (14)..(31)
  MOD_RES (42)..(42): C-terminal amidation
CDATCQFRKAIDDCYYRSRHSNVPGSVFKACMKQKKKEFKAG

SEQ ID NO: 45 - protein, 42 aa, Artificial Sequence
  Synthetic Polypeptide
  DISULFID (1)..(5)
  DISULFID (14)..(31)
  MOD_RES (42)..(42): C-terminal amidation
CDATCQFRKAIDDCYYRSHHSNVPGSVFKACMKQKKKEFKAG

SEQ ID NO: 46 - protein, 42 aa, Artificial Sequence
  Synthetic Polypeptide
  DISULFID (1)..(5)
  DISULFID (14)..(31)
  MOD_RES (42)..(42): C-terminal amidation
CDATCQYRKGLVACLYKKVAMQKRYSVFKACMKQKKKEFKAG

SEQ ID NO: 47 - protein, 43 aa, Artificial Sequence
  Synthetic Polypeptide
  DISULFID (1)..(5)
  DISULFID (14)..(31)
CDATCQFRKAIDDCYKQAHHSNVPGSVFKACMKQKKKEFKAGH

SEQ ID NO: 48 - protein, 43 aa, Artificial Sequence
  Synthetic Polypeptide
  DISULFID (1)..(5)
  DISULFID (14)..(31)
CDATCQFRKAIDDCVKQAHHSNVPGSVFKACMKQKKKEFKAGY

SEQ ID NO: 49-50 - skipped (2 entries)

SEQ ID NO: 51 - protein, 45 aa, Artificial Sequence
  Synthetic Polypeptide
  MOD_RES (1)..(1): Xaa = propargylglycine
  DISULFID (2)..(6)
  DISULFID (15)..(33)
  MOD_RES (26)..(26): Xaa = propargylglycine
XCDATCQFRKAIDDCQKQAHHSNVPXNSVFKECMKQKKKEFKAGK

SEQ ID NO: 52 - protein, 45 aa, Artificial Sequence
  Synthetic Polypeptide
  MOD_RES (1)..(1): Xaa = propargylglycine
  DISULFID (2)..(6)
  DISULFID (15)..(33)
XCDATCQFRKAIDDCQKQAHHSNVPGNSVFKECMKQKKKEFKAGK

SEQ ID NO: 53 - protein, 44 aa, Artificial Sequence
  Synthetic Polypeptide
  DISULFID (1)..(5)
  DISULFID (14)..(32)
  MOD_RES (25)..(25): Xaa = propargylglycine
CDATCQFRKAIDDCQKQAHHSNVPXNSVFKECMKQKKKEFKAGK

SEQ ID NO: 54 - protein, 42 aa, Artificial Sequence
  Synthetic Polypeptide
  DISULFID (1)..(5)
  DISULFID (14)..(31)
  MOD_RES (42)..(42): C-terminal amidation
CDATCQFRKAIDDCYWQAIHANVPGSVWKACMKFRFNVWKAG

SEQ ID NO: 55 - protein, 42 aa, Artificial Sequence
  Synthetic Polypeptide
  DISULFID (1)..(5)
  DISULFID (14)..(31)
  MOD_RES (42)..(42): C-terminal amidation
CDATCQFRKAIDDCFYQAWHSNVPGSVWKACMKFRFNVWKAG

SEQ ID NO: 56 - protein, 43 aa, Artificial Sequence
  Synthetic Polypeptide
  DISULFID (1)..(5)
  DISULFID (14)..(31)
CDATCQFRKAIDDCAKQAHHSNVPGSVFKACMKQKKKEFKAGY

SEQ ID NO: 57 - protein, 43 aa, Artificial Sequence
  Synthetic Polypeptide
  DISULFID (1)..(5)
  DISULFID (14)..(31)
CDATCQFRKAIDDCAKQAHHSNVPGSVFKACMKQKKKEFKAGH

SEQ ID NO: 58 - protein, 44 aa, Artificial Sequence
  Synthetic Polypeptide
  DISULFID (2)..(6)
  DISULFID (15)..(32)
GCDATCQFRKAIDDCAKQAHHSNVPGSVFKACMKQKKKEFKAGY

SEQ ID NO: 59 - protein, 44 aa, Artificial Sequence
  Synthetic Polypeptide
  DISULFID (2)..(6)
  DISULFID (15)..(32)
GCDATCQFRKAIDDCAKQAHHSNVPGSVFKACMKQKKKEFKAGH

SEQ ID NO: 60 - protein, 42 aa, Artificial Sequence
  Synthetic Polypeptide
  DISULFID (1)..(5)
  DISULFID (14)..(31)
  MOD_RES (42)..(42): C-terminal amidation
CDATCQFRKAIDDCYYRSWHANVPGSVFKACMKQKKKEWKAG

SEQ ID NO: 61 - protein, 38 aa, Artificial Sequence
  Synthetic Polypeptide
  DISULFID (1)..(5)
  DISULFID (14)..(27)
  MOD_RES (38)..(38): C-terminal amidation
CDATCQFRKAIDDCYYRSWHSSVFKACMKQKKKEWKAG

SEQ ID NO: 62 - protein, 43 aa, Artificial Sequence
  Synthetic Polypeptide
  DISULFID (1)..(5)
  DISULFID (14)..(31)
CDATCQFRKAIDDCYYRSWHANVPGSVFKACMKQKKKEWKAGN

SEQ ID NO: 63 - protein, 37 aa, Artificial Sequence
  Synthetic Polypeptide
  DISULFID (1)..(5)
  DISULFID (14)..(26)
  MOD_RES (37)..(37): C-terminal amidation
CDATCQFRKAIDDCYYRSWHSSFKACMKQKKKEFKAG

SEQ ID NO: 64 - protein, 42 aa, Artificial Sequence
  Synthetic Polypeptide
  DISULFID (1)..(5)
  DISULFID (14)..(31)
CDATCQFRKAIDDCYYRSWHSNVPGSVFKACMKQKKKEFKAG

SEQ ID NO: 65 - protein, 38 aa, Artificial Sequence
  Synthetic Polypeptide
  DISULFID (1)..(5)
  DISULFID (14)..(27)
  MOD_RES (38)..(38): C-terminal amidation
CDATCQFRKAIDDCARQAYHSSVFKACMKQKKKEWKAG

SEQ ID NO: 66 - protein, 43 aa, Artificial Sequence
  Synthetic Polypeptide
  DISULFID (1)..(5)
  DISULFID (14)..(31)
CDATCQFRKAIDDCYYRSWHANVPGSVFKACMKQKKKEWKAGY

SEQ ID NO: 67 - protein, 42 aa, Artificial Sequence
  Synthetic Polypeptide
  DISULFID (1)..(5)
  DISULFID (14)..(31)
  MOD_RES (42)..(42): C-terminal amidation
CDATCQFRKAIDDCYYRSWHSNVPGSVFKACMKFRFNVWKAG

SEQ ID NO: 68 - protein, 42 aa, Artificial Sequence
  Synthetic Polypeptide
  DISULFID (1)..(5)
  DISULFID (14)..(31)
CDATCQFRKAIDDCQKQAHHSNVPGSVFKACMKQKKKEFKAR

SEQ ID NO: 69 - protein, 42 aa, Artificial Sequence
  Synthetic Polypeptide
  DISULFID (1)..(5)
  DISULFID (14)..(31)
  MOD_RES (42)..(42): C-terminal amidation
CDATCQFRKAIDDCYYRSWHSNVPGSVFKACMKQRKKRWLAG

SEQ ID NO: 70 - protein, 42 aa, Artificial Sequence
  Synthetic Polypeptide
  DISULFID (1)..(5)
  DISULFID (14)..(31)
  MOD_RES (42)..(42): C-terminal amidation
CDATCFFRKVIDDCYYRSWHSNVPGSVFKACMKQLKKRWQAG

SEQ ID NO: 71 - protein, 42 aa, Artificial Sequence
  Synthetic Polypeptide
  DISULFID (1)..(5)
  DISULFID (14)..(31)
  MOD_RES (42)..(42): C-terminal amidation
CDATCHFRKAIDDCYYRSWHSNVPGSVFKACMKQHKKRWRAG

SEQ ID NO: 72 - protein, 39 aa, Artificial Sequence
  Synthetic Polypeptide
  DISULFID (1)..(5)
  DISULFID (14)..(27)
CDATCQFRKAIDDCYYRSWHSSVFKACMKQKKKEWKAGH

SEQ ID NO: 73 - protein, 42 aa, Artificial Sequence
  Synthetic Polypeptide
  DISULFID (1)..(5)
  DISULFID (14)..(31)
  MOD_RES (42)..(42): C-terminal amidation
CDATCQFRKAIDDCWIVAWHSNVPGSVFKACMKQKKKEFKAG

SEQ ID NO: 74 - protein, 42 aa, Artificial Sequence
  Synthetic Polypeptide
  DISULFID (1)..(5)
  DISULFID (14)..(31)
  MOD_RES (42)..(42): C-terminal amidation
CDATCQFRKAIDDCFTWAWHSNVPGSVFKACMKQKKKEFKAG

SEQ ID NO: 75 - protein, 39 aa, Artificial Sequence
  Synthetic Polypeptide
  DISULFID (1)..(5)
  DISULFID (14)..(27)
CDATCQFRKAIDDCVRQAHHSSVFKACMKQKKKEWKAGH

SEQ ID NO: 76 - protein, 42 aa, Artificial Sequence
  Synthetic Polypeptide
  DISULFID (1)..(5)
  DISULFID (14)..(31)
  MOD_RES (42)..(42): C-terminal amidation
CDATCQFRKAIDDCHLLAWHSNVPGSVFKACMKQKKKEFKAG

SEQ ID NO: 77 - protein, 42 aa, Artificial Sequence
  Synthetic Polypeptide
  DISULFID (1)..(5)
  DISULFID (14)..(31)
  MOD_RES (42)..(42): C-terminal amidation
CDATCQFRKAIDDCYYRSWHSNVPGSVFKACMKQKKKEWKAG

SEQ ID NO: 78 - protein, 42 aa, Artificial Sequence
  Synthetic Polypeptide
  DISULFID (1)..(5)
  DISULFID (14)..(31)
  MOD_RES (42)..(42): C-terminal amidation
CDATCQFRKAIDDCYYYAMHSNVPGSVWKACLKQKKKEFKAG

SEQ ID NO: 79 - protein, 42 aa, Artificial Sequence
  Synthetic Polypeptide
  DISULFID (1)..(5)
  DISULFID (14)..(31)
  MOD_RES (42)..(42): C-terminal amidation
CDATCQFRKAIDDCVRQAHHSNVPGSVFKACMKQKKKEWKAG

SEQ ID NO: 80 - protein, 42 aa, Artificial Sequence
  Synthetic Polypeptide
  DISULFID (1)..(5)
  DISULFID (14)..(31)
  MOD_RES (42)..(42): C-terminal amidation
CDATCQFRKAIDDCWKQAHHSNVPGSVFKACMKQKKKEFKAG

SEQ ID NO: 81 - protein, 42 aa, Artificial Sequence
  Synthetic Polypeptide
  DISULFID (1)..(5)
  DISULFID (14)..(31)
CDATCQFRKAIDDCDRQAHHSNVPGSVFKACMKQKKKEWKAG

SEQ ID NO: 82 - protein, 42 aa, Artificial Sequence; identical to SEQ ID NO: 79
  Synthetic Polypeptide
  DISULFID (1)..(5)
  DISULFID (14)..(31)

SEQ ID NO: 83 - protein, 42 aa, Artificial Sequence
  Synthetic Polypeptide
  DISULFID (1)..(5)
  DISULFID (14)..(31)
  MOD_RES (42)..(42): C-terminal amidation
CDATCQFRKAIDDCVYSAWHSNVPGSVFKACMKQKKKEFKAG

SEQ ID NO: 84 - protein, 43 aa, Artificial Sequence
  Synthetic Polypeptide
  DISULFID (1)..(5)
  DISULFID (14)..(31)
CDATCQFRKAIDDCVRQAYHSNVPGSVFKACMKQKKKEWKAGH

SEQ ID NO: 85 - protein, 42 aa, Artificial Sequence
  Synthetic Polypeptide
  DISULFID (1)..(5)
  DISULFID (14)..(31)
  MOD_RES (42)..(42): C-terminal amidation
CDATCQFRKAIDDCLLRAWHSNVPGSVFKACMKQKKKEFKAG

SEQ ID NO: 86 - protein, 43 aa, Artificial Sequence
  Synthetic Polypeptide
  DISULFID (1)..(5)
  DISULFID (14)..(31)
CDATCQFRKAIDDCVRQAHHSNVPGSVFKACMKQKKKEWKAGY

SEQ ID NO: 87 - protein, 42 aa, Artificial Sequence
  Synthetic Polypeptide
  DISULFID (1)..(5)
  DISULFID (14)..(31)
CDATCQFRKAIDDCVRQAHHSNVPGSVFKACMKQKKKEWKAN

SEQ ID NO: 88 - protein, 44 aa, Artificial Sequence
  Synthetic Polypeptide
  DISULFID (2)..(6)
  DISULFID (15)..(32)
GCDATCQFRKAIDDCVRQAHHSNVPGSVFKACMKQKKKEWKAGH

SEQ ID NO: 89 - protein, 42 aa, Artificial Sequence
  Synthetic Polypeptide
  DISULFID (1)..(5)
  DISULFID (14)..(31)
  MOD_RES (42)..(42): C-terminal amidation
CDATCQFRKAIDDCQKQAHHSNVPGSVFKACMKFRRTLWKAG

SEQ ID NO: 90 - protein, 42 aa, Artificial Sequence
  Synthetic Polypeptide
  DISULFID (1)..(5)
  DISULFID (14)..(31)
  MOD_RES (42)..(42): C-terminal amidation
CDATCQFRKAIDDCAWFAMHSNVPGSVFKACMKQKKKEFKAG

SEQ ID NO: 91 - protein, 42 aa, Artificial Sequence
  Synthetic Polypeptide
  DISULFID (1)..(5)
  DISULFID (14)..(31)
  MOD_RES (42)..(42): C-terminal amidation
CDATCQFRKAIDDCAWFALHSNVPGSVFKACMKQKKKEFKAG

SEQ ID NO: 92 - protein, 42 aa, Artificial Sequence
  Synthetic Polypeptide
  DISULFID (1)..(5)
  DISULFID (14)..(31)
  MOD_RES (42)..(42): C-terminal amidation
CDATCQFRKAIDDCWMLSWHANVPGSVFKACMKQKKKEFKAG

SEQ ID NO: 93 - protein, 42 aa, Artificial Sequence
  Synthetic Polypeptide
  DISULFID (1)..(5)
  DISULFID (14)..(31)
  MOD_RES (42)..(42): C-terminal amidation
CDATCQFRKAIDDCQKQAHHSNVPGSVFKACVLQKKKEFKAG

SEQ ID NO: 94 - protein, 43 aa, Artificial Sequence
  Synthetic Polypeptide
  DISULFID (1)..(5)
  DISULFID (14)..(31)
CDATCQFRKAIDDCVKQAHHSNVPGSVFKACMKQKKKEFKAGH

SEQ ID NO: 95 - protein, 42 aa, Artificial Sequence
  Synthetic Polypeptide
  DISULFID (1)..(5)
  DISULFID (14)..(31)
CDATCQFRKAIDDCQKQAHHSNVPGSVFKACMKQKKKEFKAW

SEQ ID NO: 96 - protein, 42 aa, Artificial Sequence
  Synthetic Polypeptide
  DISULFID (1)..(5)
  DISULFID (14)..(31)
CDATCQFRKAIDDCQKQAHHSNVPGSVFKACMKQKKKEFKAQ

SEQ ID NO: 97 - protein, 42 aa, Artificial Sequence
  Synthetic Polypeptide
  DISULFID (1)..(5)
  DISULFID (14)..(31)
  MOD_RES (30)..(30): Xaa = 2-aminoisobutyric acid
  MOD_RES (42)..(42): C-terminal amidation
CDATCQFRKAIDDCQKQEHHSNVPGSKFKXCMKQKKKEFKAG

SEQ ID NO: 98 - protein, 42 aa, Artificial Sequence
  Syntehtic Polypeptide
  DISULFID (1)..(5)
  DISULFID (14)..(31)
  MOD_RES (30)..(30): Xaa = 2-aminoisobutyric acid
  MOD_RES (42)..(42): C-terminal amidation
CDATCQFRKAIDDCQKQAHHSNVPGSVFKXCMKQKKKEFKAA

SEQ ID NO: 99 - protein, 42 aa, Artificial Sequence
  Synthetic Polypeptide
  DISULFID (1)..(5)
  DISULFID (14)..(31)
CDATCQFRKAIDDCVRQAHHSNVPGSVFKACMKQKKKEWKAH

SEQ ID NO: 100 - protein, 42 aa, Artificial Sequence
  Synthetic Polypeptide
  DISULFID (1)..(5)
  DISULFID (14)..(31)
  MOD_RES (42)..(42): C-terminal amidation
CDATCQFRKAIDDCQKQAHHSNVPGSVFKACLLQKKKEFKAG

SEQ ID NO: 101 - protein, 42 aa, Artificial Sequence
  Synthetic Polypeptide
  DISULFID (1)..(5)
  DISULFID (14)..(31)
  MOD_RES (42)..(42): C-terminal amidation
CDATCQFRKAIDDCQKQAHHSNVPGSVFKACLVQKKKEFKAG

SEQ ID NO: 102 - protein, 42 aa, Artificial Sequence
  Synthetic Polypeptide
  DISULFID (1)..(5)
  DISULFID (14)..(31)
  MOD_RES (42)..(42): C-terminal amidation
CDATCQFRKAIDDCQKQAHHSNVPGSVFKACMVQKKKEFKAG

SEQ ID NO: 103 - protein, 42 aa, Artificial Sequence
  Synthetic Polypeptide
  DISULFID (1)..(5)
  DISULFID (14)..(31)
  MOD_RES (42)..(42): C-terminal amidation
CDATCQFRKAIDDCQKQAHHSNVPGSVFKACMLQKKKEFKAG

SEQ ID NO: 104 - protein, 42 aa, Artificial Sequence
  Synthetic Polypeptide
  DISULFID (1)..(5)
  DISULFID (14)..(31)
  MOD_RES (42)..(42): C-terminal amidation
CDATCQFRKAIDDCYYRAWHSNVPGSVFKACMKQKKKEFKAG

SEQ ID NO: 105 - protein, 43 aa, Artificial Sequence
  Synthetic Polypeptide
  DISULFID (1)..(5)
  DISULFID (14)..(31)
CDATCQFRKAIDDCARQAHHSNVPGSVWKACMKQKKKEWKAGH

SEQ ID NO: 106 - protein, 43 aa, Artificial Sequence
  Synthetic Polypeptide
  DISULFID (1)..(5)
  DISULFID (14)..(31)
CDATCQFRKAIDDCVRQAHHSNVPGSVWKACMKQKKKEWKAGH

SEQ ID NO: 107 - protein, 43 aa, Artificial Sequence
  Synthetic Polypeptide
  DISULFID (1)..(5)
  DISULFID (14)..(31)
CDATCQFRKAIDDCFTWSWHSNVPGSVFKACMKQKKKEFKAGH

SEQ ID NO: 108 - protein, 43 aa, Artificial Sequence
  Synthetic Polypeptide
  DISULFID (1)..(5)
  DISULFID (14)..(31)
CDATCQFRKAIDDCYWQAIHANVPGSVWKACMKQKKKEFKAGH

SEQ ID NO: 109 - protein, 43 aa, Artificial Sequence
  Synthetic Polypeptide
  DISULFID (1)..(5)
  DISULFID (14)..(31)
CDATCQFRKAIDDCFYQAWHSNVPGSVWKACMKQKKKEFKAGH

SEQ ID NO: 110 - protein, 43 aa, Artificial Sequence
  Synthetic Polypeptide
  DISULFID (1)..(5)
  DISULFID (14)..(31)
CDATCQFRKAIDDCVWFAWHSNVPGSVFKACMKQKKKEFKAGH

SEQ ID NO: 111 - protein, 43 aa, Artificial Sequence
  Synthetic Polypeptide
  DISULFID (1)..(5)
  DISULFID (14)..(31)
CDATCQFRKAIDDCWMLSWHANVPGSVFKACMKQKKKEFKAGH

SEQ ID NO: 112 - protein, 43 aa, Artificial Sequence
  Synthetic Polypeptide
  DISULFID (1)..(5)
  DISULFID (14)..(31)
CDATCQFRKAIDDCYYRSWHSNVPGSVFKACMKQKKKEFKAGH

SEQ ID NO: 113 - protein, 42 aa, Artificial Sequence
  Synthetic Polypeptide
  DISULFID (1)..(5)
  DISULFID (14)..(31)
  MOD_RES (42)..(42): C-terminal amidation
CDATCQFRKAIDDCQKQAHHSNVPGSVFKACMKRRRLLWKAG

SEQ ID NO: 114 - protein, 42 aa, Artificial Sequence
  Synthetic Polypeptide
  DISULFID (1)..(5)
  DISULFID (14)..(31)
  MOD_RES (42)..(42): C-terminal amidation
CDATCQFRKAIDDCQKQAHHSNVPGSVFKACMKERRRRWKAG

SEQ ID NO: 115 - protein, 42 aa, Artificial Sequence
  Synthetic Polypeptide
  DISULFID (1)..(5)
  DISULFID (14)..(31)
  MOD_RES (42)..(42): C-terminal amidation
CDATCQFRKAIDDCSWFAIHSNVPGSVFKACMKQKKKEFKAG

SEQ ID NO: 116 - protein, 42 aa, Artificial Sequence
  Synthetic Polypeptide
  DISULFID (1)..(5)
  DISULFID (14)..(31)
  MOD_RES (42)..(42)
CDATCQFRKAIDDCMWYAYHSNVPGSVFKACMKQKKKEFKAG

SEQ ID NO: 117 - protein, 42 aa, Artificial Sequence
  Synthetic Polypeptide
  DISULFID (1)..(5)
  DISULFID (14)..(31)
  MOD_RES (42)..(42): C-terminal amidation
CDATCQFRKAIDDCLWWSQHSNVPGSVFKACMKQKKKEFKAG

SEQ ID NO: 118 - protein, 42 aa, Artificial Sequence
  Synthetic Polypeptide
  DISULFID (1)..(5)
  DISULFID (14)..(31)
  MOD_RES (42)..(42): C-terminal amidation
CDATCQFRKAIDDCVWKAFHANVPGSVFKACMKQKKKEFKAG

SEQ ID NO: 119 - protein, 42 aa, Artificial Sequence
  Synthetic Polypeptide
  DISULFID (1)..(5)
  DISULFID (14)..(31)
  MOD_RES (42)..(42): C-terminal amidation
CDATCQFRKAIDDCFWLASHSNVPGSVWKACMKQKKKEFKAG

SEQ ID NO: 120 - protein, 42 aa, Artificial Sequence
  Synthetic Polypeptide
  DISULFID (1)..(5)
  DISULFID (14)..(31)
  MOD_RES (42)..(42): C-terminal amidation
CDATCQFRKAIDDCLWYARHSNVPGSVFKACMKQKKKEFKAG

SEQ ID NO: 121 - protein, 42 aa, Artificial Sequence
  Synthetic Polypeptide
  DISULFID (1)..(5)
  DISULFID (14)..(31)
  MOD_RES (42)..(42): C-terminal amidation
CDATCQFRKAIDDCMWYSRHSNVPGSVFKACMKQKKKEFKAG

SEQ ID NO: 122 - protein, 42 aa, Artificial Sequence
  Synthetic Polypeptide
  DISULFID (1)..(5)
  DISULFID (14)..(31)
  MOD_RES (42)..(42): C-terminal amidation
CDATCQFRKAIDDCMWFAWHSNVPGSVFKACMKQKKKEFKAG

SEQ ID NO: 123 - protein, 42 aa, Artificial Sequence
  Synthetic Polypeptide
  DISULFID (1)..(5)
  DISULFID (14)..(31)
  MOD_RES (42)..(42): C-terminal amidation
CDATCQFRKAIDDCIFWAAHSNVPGSVFKACMKQKKKEFKAG

SEQ ID NO: 124 - protein, 42 aa, Artificial Sequence
  Synthetic Polypeptide
  DISULFID (1)..(5)
  DISULFID (14)..(31)
  MOD_RES (42)..(42): C-terminal amidation
CDATCHFRKAIDDCQKQAHHSNVPGSVFKACMKQHKKRWRAG

SEQ ID NO: 125 - protein, 42 aa, Artificial Sequence
  Synthetic Polypeptide
  DISULFID (1)..(5)
  DISULFID (14)..(31)
  MOD_RES (42)..(42): C-terminal amidation
CDATCFFRKVIDDCQKQAHHSNVPGSVFKACMKQLKKRWQAG

SEQ ID NO: 126 - protein, 42 aa, Artificial Sequence
  Synthetic Polypeptide
  DISULFID (1)..(5)
  DISULFID (14)..(31)
  MOD_RES (42)..(42): C-terminal amidation
CDATCQFRKAIDDCQKQAHHSNVPGSVFKACMKQRKKRWLAG

SEQ ID NO: 127 - protein, 42 aa, Artificial Sequence
  Synthetic Polypeptide
  DISULFID (1)..(5)
  DISULFID (14)..(31)
  MOD_RES (42)..(42): C-terminal amidation
CDATCQFRKAIDDCQKQAHHSNVPGSVFKACMKFRFNVWKAG

SEQ ID NO: 128 - protein, 42 aa, Artificial Sequence
  Synthetic Polypeptide
  DISULFID (1)..(5)
  DISULFID (14)..(31)
  MOD_RES (42)..(42): C-terminal amidation
CDATCQFRKAIDDCQKQAHHSNVPGSVFKACMKFRRFLWKAG

SEQ ID NO: 129 - protein, 42 aa, Artificial Sequence
  Synthetic Polypeptide
  DISULFID (1)..(5)
  DISULFID (14)..(31)
  MOD_RES (42)..(42): C-terminal amidation
CDATCQFRKAIDDCWIVAWHANVPGSVFKACMKQKKKEFKAG

SEQ ID NO: 130 - protein, 42 aa, Artificial Sequence
  Synthetic Polypeptide
  DISULFID (1)..(5)
  DISULFID (14)..(31)
  MOD_RES (42)..(42): C-terminal amidation
CDATCQFRKAIDDCWVIAWHSNVPGSVFKACMKQKKKEFKAG

SEQ ID NO: 131 - protein, 42 aa, Artificial Sequence
  Synthetic Polypeptide
  DISULFID (1)..(5)
  DISULFID (14)..(31)
  MOD_RES (42)..(42): C-terminal amidation
CDATCQFRKAIDDCMLFSWHSNVPGSVFKACMKQKKKEFKAG

SEQ ID NO: 132 - protein, 42 aa, Artificial Sequence
  Synthetic Polypeptide
  DISULFID (1)..(5)
  DISULFID (14)..(31)
  MOD_RES (42)..(42): C-terminal amidation
CDATCQFRKAIDDCMLLSWHSNVPGSVFKACMKQKKKEFKAG

SEQ ID NO: 133 - protein, 42 aa, Artificial Sequence
  Synthetic Polypeptide
  DISULFID (1)..(5)
  DISULFID (14)..(31)
  MOD_RES (42)..(42): C-terminal amidation
CDATCQFRKAIDDCVWYSMHSNVPGSVFKACMKQKKKEFKAG

SEQ ID NO: 134 - protein, 42 aa, Artificial Sequence
  Synthetic Polypeptide
  DISULFID (1)..(5)
  DISULFID (14)..(31)
  MOD_RES (42)..(42): C-terminal amidation
CDATCQFRKAIDDCWVQAWHSNVPGSVFKACMKQKKKEFKAG

SEQ ID NO: 135 - protein, 42 aa, Artificial Sequence
  Synthetic Polyppeptide
  DISULFID (1)..(5)
  DISULFID (14)..(31)
  MOD_RES (42)..(42): C-terminal amidation
CDATCQFRKAIDDCFTWSWHSNVPGSVFKACMKQKKKEFKAG

SEQ ID NO: 136 - protein, 42 aa, Artificial Sequence
  Synthetic Polypeptide
  DISULFID (1)..(5)
  DISULFID (14)..(31)
  MOD_RES (42)..(42): C-terminal amidation
CDATCQFRKAIDDCVFWAAHSNVPGSVFKACMKQKKKEFKAG

SEQ ID NO: 137 - protein, 42 aa, Artificial Sequence
  Synthetic Polypeptide
  DISULFID (1)..(5)
  DISULFID (14)..(31)
  MOD_RES (42)..(42): C-terminal amidation
CDATCQFRKAIDDCVYSAWHANVPGSVFKACMKQKKKEFKAG

SEQ ID NO: 138 - protein, 42 aa, Artificial Sequence
  Synthetic Polypeptide
  DISULFID (1)..(5)
  DISULFID (14)..(31)
  MOD_RES (42)..(42): C-terminal amidation
CDATCQFRKAIDDCYWQAIHANVPGSVWKACMKQKKKEFKAG

SEQ ID NO: 139 - protein, 42 aa, Artificial Sequence
  Synthetic Polypeptide
  DISULFID (1)..(5)
  DISULFID (14)..(31)
  MOD_RES (42)..(42): C-terminal amidation
CDATCQFRKAIDDCFYQAWHSNVPGSVWKACMKQKKKEFKAG

SEQ ID NO: 140 - protein, 42 aa, Artificial Sequence
  Synthetic Polypeptide
  DISULFID (1)..(5)
  DISULFID (14)..(31)
  MOD_RES (42)..(42): C-terminal amidation
CDATCQFRKAIDDCHLLAWHANVPGSVFKACMKQKKKEFKAG

SEQ ID NO: 141 - protein, 42 aa, Artificial Sequence
  Synthetic Polypeptide
  DISULFID (1)..(5)
  DISULFID (14)..(31)
  MOD_RES (42)..(42): C-terminal amidation
CDATCQFRKAIDDCHWYSLHSNVPGSVFKACMKQKKKEFKAG

SEQ ID NO: 142 - protein, 42 aa, Artificial Sequence
  Synthetic Polypeptide
  DISULFID (1)..(5)
  DISULFID (14)..(31)
  MOD_RES (42)..(42): C-terminal amidation
CDATCQFRKAIDDCQKQAHHSNVPGSVFKACVKQKKKEFKAG

SEQ ID NO: 143 - protein, 42 aa, Artificial Sequence
  Synthetic Polypeptide
  DISULFID (1)..(5)
  DISULFID (14)..(31)
  MOD_RES (42)..(42): C-terminal amidation
CDATCQFRKAIDDCQKQAHHSNVPGSVFKACLKQKKKEFKAG

SEQ ID NO: 144 - protein, 42 aa, Artificial Sequence
  Synthetic Polypeptide
  DISULFID (1)..(5)
  DISULFID (14)..(31)
  MOD_RES (42)..(42): C-terminal amidation
CDATCQFRKAIDDCDRQAYHSNVPGSVFKACMKQKKKEWKAG

SEQ ID NO: 145 - protein, 43 aa, Artificial Sequence
  Synthetic Polypeptide
  DISULFID (1)..(5)
  DISULFID (14)..(31)
CDATCQFRKAIDDCQKQAHHSNVPGSVFKACMKQKKKEFKAGW

SEQ ID NO: 146 - protein, 42 aa, Artificial Sequence
  Synthetic Polypeptide
  DISULFID (1)..(5)
  DISULFID (14)..(31)
  MOD_RES (42)..(42): C-terminal amidation
CDATCQFRKAIDDCQKQAHHSNVPGSVFKTCMKQKKKEFKAG

SEQ ID NO: 147 - protein, 42 aa, Artificial Sequence
  Synthetic Polypeptide
  DISULFID (1)..(5)
  DISULFID (14)..(31)
  MOD_RES (42)..(42): C-terminal amidation
CDATCQFRKAIDDCYWIAMHSNVPGSVWKACMKQKKKEFKAG

SEQ ID NO: 148 - protein, 42 aa, Artificial Sequence
  Synthetic Polypeptide
  DISULFID (1)..(5)
  DISULFID (14)..(31)
  MOD_RES (42)..(42): C-terminal amidation
CDATCQFRKAIDDCVWFAWHSNVPGSVFKACMKQKKKEFKAG

SEQ ID NO: 149 - protein, 42 aa, Artificial Sequence; identical to SEQ ID NO: 64
  Synthetic Polypeptide
  DISULFID (1)..(5)
  DISULFID (14)..(31)
  MOD_RES (42)..(42): C-terminal amidation

SEQ ID NO: 150 - protein, 42 aa, Artificial Sequence
  Synthetic Polypeptide
  DISULFID (1)..(5)
  DISULFID (14)..(31)
  MOD_RES (42)..(42): C-terminal amidation
CDATCQFRKAIDDCYYYAMHSNVPGSVWKACMKQKKKEFKAG

SEQ ID NO: 151 - protein, 43 aa, Artificial Sequence; identical to SEQ ID NO: 2
  Synthetic Polypeptide
  DISULFID (1)..(5)
  DISULFID (14)..(31)

SEQ ID NO: 152 - protein, 43 aa, Artificial Sequence
  Synthetic Polypeptide
  DISULFID (1)..(5)
  DISULFID (14)..(31)
CDATCQFRKAIDDCAKQAHHSNVPGSVFKACMKQKKKEWKAGH

SEQ ID NO: 153 - protein, 42 aa, Artificial Sequence
  Synthetic Polypeptide
  DISULFID (1)..(5)
  DISULFID (14)..(31)
CDATCQFRKAIDDCQKQAHHSNVPGSVFKACMKQKKKEFKAH

SEQ ID NO: 154 - protein, 43 aa, Artificial Sequence
  Synthetic Polypeptide
  DISULFID (1)..(5)
  DISULFID (14)..(31)
CDATCQFRKAIDDCDRQAHHSNVPGSVFKACMKQKKKEWKANN

SEQ ID NO: 155 - protein, 43 aa, Artificial Sequence
  Synthetic Polypeptide
  DISULFID (1)..(5)
  DISULFID (14)..(31)
CDATCQFRKAIDDCDRQAHHSNVPGSVFKACMKQKKKEFKAGH

SEQ ID NO: 156 - protein, 43 aa, Artificial Sequence
  Synthetic Polypeptide
  DISULFID (1)..(5)
  DISULFID (14)..(31)
CDATCQFRKAIDDCVRQAHHSNVPGSVFKACMKQKKKEWKAGH

SEQ ID NO: 157 - protein, 44 aa, Artificial Sequence
  Synthetic Polypeptide
  DISULFID (1)..(5)
  DISULFID (14)..(31)
  MOD_RES (30)..(30): Xaa = 2-aminoisobutyric acid
CDATCQFRKAIDDCQKQAHHSNVPGSVFKXCMKQKKKEFKAGGS

SEQ ID NO: 158 - protein, 42 aa, Artificial Sequence
  Synthetic Polypeptide
  DISULFID (1)..(5)
  DISULFID (14)..(31)
  MOD_RES (42)..(42): C-terminal amidation
CDATCQFRKAIDDCDRQAHHSNVPGSVFKACMKQKKKEWKAN

SEQ ID NO: 159 - protein, 42 aa, Artificial Sequence; identical to SEQ ID NO: 158
  Synthetic Polypeptide
  DISULFID (1)..(5)
  DISULFID (14)..(31)

SEQ ID NO: 160 - protein, 48 aa, Artificial Sequence
  Synthetic Polypeptide
  DISULFID (1)..(5)
  DISULFID (14)..(31)
CDATCQFRKAIDDCQKQAHHSNVPGSVFKACMKQKKKEFKAGHHHHHH

SEQ ID NO: 161 - protein, 43 aa, Artificial Sequence
  Synthetic Polypeptide
  DISULFID (1)..(5)
  DISULFID (14)..(31)
  MOD_RES (30)..(30): Xaa = 2-aminoisobutyric acid
CDATCQFRKAIDDCQKQAHHSNVPGSVFKXCMKQKKKEFKANK

SEQ ID NO: 162 - protein, 42 aa, Artificial Sequence
  Synthetic Polypeptide
  DISULFID (1)..(5)
  DISULFID (14)..(31)
  MOD_RES (30)..(30): Xaa = 2-aminoisobutyric acid
CDATCQFRKAIDDCQKQAHHSNVPGSVFKXCMKQKKKEWKAN

SEQ ID NO: 163 - protein, 42 aa, Artificial Sequence; identical to SEQ ID NO: 81
  Synthetic Polypeptide
  DISULFID (1)..(5)
  DISULFID (14)..(31)
  MOD_RES (42)..(42): C-terminal amidation

SEQ ID NO: 164 - protein, 43 aa, Artificial Sequence
  Synthetic Polypeptide
  DISULFID (1)..(5)
  DISULFID (14)..(31)
CDATCQFRKAIDDCQKQAHHSNVPGSVFKACMKQKKKEFKAGY

SEQ ID NO: 165 - skipped

SEQ ID NO: 166 - protein, 42 aa, Artificial Sequence; identical to SEQ ID NO: 162
  Synthetic Polypeptide
  DISULFID (1)..(5)
  DISULFID (14)..(31)
  MOD_RES (30)..(30): Xaa = 2-aminoisobutyric acid
  MOD_RES (42)..(42): C-terminal amidation

SEQ ID NO: 167 - protein, 43 aa, Artificial Sequence
  Synthetic Polypeptide
  DISULFID (1)..(5)
  DISULFID (14)..(31)
CDATCQFRKAIDDCDRQAHHSNVPGSVFKACMKQKKKEWKAGH

SEQ ID NO: 168 - protein, 42 aa, Artificial Sequence
  Synthetic Polypeptide
  DISULFID (1)..(5)
  DISULFID (14)..(31)
  MOD_RES (42)..(42): C-terminal amidation
CDATCQFRKAIDDCDRQAHHSNVPGSVFKACMKQKKKEFKAG

SEQ ID NO: 169 - protein, 42 aa, Artificial Sequence
  Synthetic Polypeptide
  DISULFID (1)..(5)
  DISULFID (14)..(31)
  MOD_RES (42)..(42): C-terminal amidation
CDATCQFRKAIDDCDKQAHHSNVPGSVFKACMKQKKKEFQAG

SEQ ID NO: 170 - protein, 43 aa, Artificial Sequence
  Synthetic Polypeptide
  DISULFID (1)..(5)
  DISULFID (14)..(31)
CDATCQFRKAIDDCQKQAHHSNVPGSVFKACMKQKKKEFKAGR

SEQ ID NO: 171 - protein, 43 aa, Artificial Sequence
  Synthetic Polypeptide
  DISULFID (1)..(5)
  DISULFID (14)..(31)
CDATCQFRKAIDDCQKQAHHSNVPGSVFKACMKQKKKEFKAGH

SEQ ID NO: 172 - protein, 43 aa, Artificial Sequence
  Synthetic Polypeptide
  DISULFID (1)..(5)
  DISULFID (14)..(31)
CDATCQFRKAIDDCQKQAHHSNVPGSVFKACMKQKKKEFKAGF

SEQ ID NO: 173 - protein, 43 aa, Artificial Sequence
  Synthetic Polypeptide
  DISULFID (1)..(5)
  DISULFID (14)..(31)
CDATCQFRKAIDDCQKQAHHSNVPGSVFKACMKQKKKEFKAGE

SEQ ID NO: 174 - protein, 43 aa, Artificial Sequence
  Synthetic Polypeptide
  DISULFID (1)..(5)
  DISULFID (14)..(31)
CDATCQFRKAIDDCQKQAHHSNVPGSVFKACMKQKKKEFKAGQ

SEQ ID NO: 175 - protein, 43 aa, Artificial Sequence
  Synthetic Polypeptide
  DISULFID (1)..(5)
  DISULFID (14)..(31)
CDATCQFRKAIDDCQKQAHHSNVPGSVFKACMKQKKKEFKAGA

SEQ ID NO: 176 - protein, 42 aa, Artificial Sequence
  Synthetic Polypeptide
  DISULFID (1)..(5)
  DISULFID (10)..(35)
  MOD_RES (42)..(42): C-terminal amidation
CDATCQFRKCIDDWQKQAHHSNVPGSVFKARMKQCKKEFKAG

SEQ ID NO: 177 - protein, 46 aa, Artificial Sequence
  Synthetic Polypeptide
  DISULFID (1)..(5)
  DISULFID (14)..(31)
CDATCQFRKAIDDCQKQAHHSNVPGSVFKACMKQKKKEFKAGGGGS

SEQ ID NO: 178 - protein, 37 aa, Artificial Sequence
  Synthetic Polypeptide
  DISULFID (1)..(5)
  DISULFID (14)..(26)
  DISULFID (25)..(25): Xaa = 2-aminoisobutyric acid
  MOD_RES (37)..(37): C-terminal amidation
CDATCQFRKAIDDCDKQAYHSSFKXCMKQKKKEFKAG

SEQ ID NO: 179 - protein, 42 aa, Artificial Sequence
  Synthetic Polypeptide
  DISULFID (1)..(5)
  DISULFID (14)..(31)
  MOD_RES (42)..(42): C-terminal amidation
CDATCQFRKAIDDCVKQAHHSNVPGSVFKACMKQKKKEFKAG

SEQ ID NO: 180 - protein, 42 aa, Artificial Sequence
  Synthetic Polypeptide
  DISULFID (1)..(5)
  DISULFID (14)..(31)
  MOD_RES (42)..(42): C-terminal amidation
CDATCQFRKAIDDCAKQAHHSNVPGSVFKACMKQKKKEFKAG

SEQ ID NO: 181 - protein, 43 aa, Artificial Sequence
  Synthetic Polypeptide
  DISULFID (2)..(6)
  DISULFID (15)..(32)
  MOD_RES (43)..(43): C-terminal amidation
GCDATCQFRKAIDDCQKQAHHSNVPGSVFKACMKQKKKEFKAG

SEQ ID NO: 182 - protein, 43 aa, Artificial Sequence
  Synthetic Polypeptide
  DISULFID (1)..(5)
  DISULFID (14)..(31)
CDATCQFRKAIDDCQKQAHHSNVPGSVFKACMKQKKKEFKAGK

SEQ ID NO: 183 - protein, 43 aa, Artificial Sequence
  Synthetic Polypeptide
  DISULFID (2)..(6)
  DISULFID (15)..(32)
  MOD_RES (43)..(43): C-terminal amidation
SCDATCQFRKAIDDCQKQAHHSNVPGSVFKACMKQKKKEFKAG

SEQ ID NO: 184 - protein, 43 aa, Artificial Sequence
  Synthetic Polypeptide
  DISULFID (2)..(6)
  DISULFID (15)..(32)
  MOD_RES (43)..(43): C-terminal amidation
ACDATCQFRKAIDDCQKQAHHSNVPGSVFKACMKQKKKEFKAG

SEQ ID NO: 185 - protein, 44 aa, Artificial Sequence
  Synthetic Polypeptide
  DISULFID (3)..(7)
  DISULFID (16)..(33)
  MOD_RES (44)..(44): C-terminal amidation
GSCDATCQFRKAIDDCQKQAHHSNVPGSVFKACMKQKKKEFKAG

SEQ ID NO: 186 - protein, 42 aa, Artificial Sequence
  Synthetic Polypeptide
  DISULFID (1)..(5)
  DISULFID (14)..(31)
  MOD_RES (30)..(30): Xaa = 2-aminoisobutyric acid
  MOD_RES (42)..(42): C-terminal amidation
CDATCQFRKAIDDCQKQAHHSNVPGNSFKXCMKQKKKEFKAG

SEQ ID NO: 187 - protein, 42 aa, Artificial Sequence
  Synthetic Polypeptide
  DISULFID (1)..(5)
  DISULFID (14)..(31)
  MOD_RES (30)..(30): Xaa = 2-aminoisobutyric acid
  MOD_RES (39)..(39): Xaa = para-iodophenyalanine
  MOD_RES (42)..(42): C-terminal amidation
CDATCQFRKAIDDCQKQAHHSNVPGSVFKXCMKQKKKEXKAG

SEQ ID NO: 188 - protein, 42 aa, Artificial Sequence
  Synthetic Polypeptide
  DISULFID (1)..(5)
  DISULFID (14)..(31)
  MOD_RES (24)..(24): Xaa = 3,4-Dehydro-Proline
  MOD_RES (30)..(30): Xaa = 2-aminoisobutyric acid
  MOD_RES (42)..(42): C-terminal amidation
CDATCQFRKAIDDCQKQAHHSNVXGSVFKXCMKQKKKEFKAG

SEQ ID NO: 189 - protein, 43 aa, Artificial Sequence
  Synthetic Polypeptide
  DISULFID (1)..(5)
  DISULFID (14)..(32)
  MOD_RES (31)..(31): Xaa = 2-aminoisobutyric acid
  MOD_RES (43)..(43): C-terminal amidation
CDATCQFRKAIDDCQKQAHHSNVPGNSVFKXCMKQKKKEFKAG

SEQ ID NO: 190 - protein, 42 aa, Artificial Sequence
  Synthetic Polypeptide
  DISULFID (1)..(5)
  DISULFID (14)..(31)
CDATCQFRKAIDDCQKQAHHSNVPGSVFKACMKQKKKEFKAG

SEQ ID NO: 191 - protein, 42 aa, Artificial Sequence
  Synthetic Polypeptide
  DISULFID (1)..(5)
  DISULFID (14)..(31)
  MOD_RES (30)..(30): Xaa = 2-aminoisobutyric acid
  MOD_RES (42)..(42): C-terminal amidation
CDATCQFRKAIDDCQKQAHHSNEPGSVFKXCMKQKKKEFKAG

SEQ ID NO: 192 - protein, 42 aa, Artificial Sequence
  Synthetic Polypeptide
  DISULFID (1)..(5)
  DISULFID (14)..(31)
  MOD_RES (30)..(30): Xaa = 2-aminoisobutyric acid
  MOD_RES (42)..(42): C-terminal amidation
CDATCQFRKAIDDCQKQAHHSEVPGSVFKXCMKQKKKEFKAG

SEQ ID NO: 193 - protein, 42 aa, Artificial Sequence
  Synthetic Polypeptide
  DISULFID (1)..(5)
  DISULFID (14)..(31)
  MOD_RES (30)..(30): Xaa = 2-aminoisobutyric acid
  MOD_RES (42)..(42): C-terminal amidation
CDATCQFRKAIDDCQKQAHHSNVPNSVFKXCMKQKKKEFKAG

SEQ ID NO: 194 - protein, 42 aa, Artificial Sequence
  Synthetic Polypeptide
  DISULFID (1)..(5)
  DISULFID (14)..(31)
  MOD_RES (30)..(30): Xaa = 2-aminoisobutyric acid
  MOD_RES (42)..(42): C-terminal amidation
CDATCQFRKAIDDCQKQAHHSNVGNSVFKXCMKQKKKEFKAG

SEQ ID NO: 195-196 - skipped (2 entries)

SEQ ID NO: 197 - protein, 47 aa, Artificial Sequence
  Synthetic Polypeptide
  DISULFID (1)..(5)
  DISULFID (14)..(36)
  MOD_RES (35)..(35): Xaa = 2-aminoisobutyric acid
  MOD_RES (47)..(47): C-terminal amidation
CDATCQFRKAIDDCQKQAHHSNVPGLQTSVSVFKXCMKQKKKEFKAG

SEQ ID NO: 198 - protein, 42 aa, Artificial Sequence
  Synthetic Polypeptide
  DISULFID (1)..(5)
  DISULFID (14)..(31)
  MOD_RES (26)..(26): Xaa = 2-aminoisobutyric acid
  MOD_RES (30)..(30): Xaa = 2-aminoisobutyric acid
  MOD_RES (42)..(42): C-terminal amidation
CDATCQFRKAIDDCQKQAHHSNVPGXVFKXCMKQKKKEFKAG

SEQ ID NO: 199 - protein, 48 aa, Artificial Sequence
  Synthetic Polypeptide
  DISULFID (2)..(6)
  DISULFID (15)..(32)
MCDATCQFRKAIDDCQKQAHHSNVPGSVFKACMKQKKKEFKAGHHHHH

SEQ ID NO: 200 - protein, 42 aa, Artificial Sequence
  Synthetic Polypeptide
  DISULFID (1)..(5)
  DISULFID (14)..(31)
  MOD_RES (30)..(30): Xaa = 2-aminoisobutyric acid
  MOD_RES (42)..(42): C-terminal amidation
CDATCQFRKAIDDCQKQAHHSNVPGDVFKXCMKQKKKEFKAG

SEQ ID NO: 201 - protein, 41 aa, Artificial Sequence
  Synthetic Polypeptide
  DISULFID (1)..(5)
  DISULFID (14)..(30)
  MOD_RES (29)..(29): Xaa = 2-aminoisobutyric acid
  MOD_RES (41)..(41): C-terminal amidation
CDATCQFRKAIDDCDKQAYHSNVPGSFKXCMKQKKKEFKAG

SEQ ID NO: 202 - protein, 42 aa, Artificial Sequence
  Synthetic Polypeptide
  DISULFID (1)..(5)
  DISULFID (14)..(31)
CDATCQFRKAIDDCQKQAHHSNVPGSVFKACMKQKKKEFKAN

SEQ ID NO: 203 - protein, 42 aa, Artificial Sequence
  Synthetic Polypeptide
  DISULFID (1)..(5)
  DISULFID (14)..(31)
  MOD_RES (30)..(30): Xaa = 2-aminoisobutyric acid
  MOD_RES (42)..(42): C-terminal amidation
CDATCQFRKAIEDCQKQAHHSNVPGSVFKXCMKQKKKEFKAG

SEQ ID NO: 204 - protein, 49 aa, Artificial Sequence
  Synthetic Polypeptide
  DISULFID (2)..(6)
  DISULFID (15)..(32)
MCDATCQFRKAIDDCQKQAHHSNVPGSVFKACMKQKKKEFKAGHHHHHH

SEQ ID NO: 205 - protein, 42 aa, Artificial Sequence; identical to SEQ ID NO: 202
  Synthetic Polypeptide
  DISULFID (1)..(5)
  DISULFID (14)..(31)
  MOD_RES (42)..(42): C-terminal amidation

SEQ ID NO: 206 - protein, 42 aa, Artificial Sequence
  Synthetic Polypeptide
  DISULFID (1)..(5)
  DISULFID (14)..(31)
  MOD_RES (30)..(30): Xaa = 2-aminoisobutyric acid
CDATCQFRKAIDDCQKQAHHSNVPGSVFKXCMKQKKKEFKAN

SEQ ID NO: 207 - protein, 42 aa, Artificial Sequence
  Synthetic Polypeptide
  DISULFID (1)..(5)
  DISULFID (14)..(31)
  MOD_RES (42)..(42): C-terminal amidation
CDATCQFRKAIDDCQKQAHHSNVPGSVFKSCMKQKKKEFKAG

SEQ ID NO: 208 - protein, 42 aa, Artificial Sequence
  Synthetic Polypeptide
  DISULFID (1)..(5)
  DISULFID (14)..(31)
  MOD_RES (30)..(30): Xaa = 2-aminoisobutyric acid
  MOD_RES (42)..(42): C-terminal amidation
CDATCQFRKAIDDCQKQAHHSNVPGNVFKXCMKQKKKEFKAG

SEQ ID NO: 209 - protein, 42 aa, Artificial Sequence
  Synthetic Popypeptide
  DISULFID (1)..(5)
  DISULFID (14)..(31)
  MOD_RES (30)..(30): Xaa = 2-aminoisobutyric acid
  MOD_RES (42)..(42): C-terminal amidation
CDATCQFRKAIDDCQKQAHHSNVPGGVFKXCMKQKKKEFKAG

SEQ ID NO: 210 - protein, 42 aa, Artificial Sequence; identical to SEQ ID NO: 209
  Synthetic Polypeptide
  DISULFID (1)..(41)
  MOD_RES (30)..(30): Xaa = 2-aminoisobutyric acid
  MOD_RES (42)..(42): C-terminal amidation

SEQ ID NO: 211 - protein, 42 aa, Artificial Sequence
  Synthetic Polypeptide
  DISULFID (1)..(5)
  DISULFID (14)..(31)
  MOD_RES (42)..(42): C-terminal amidation
CDATCQFRKAIDDCQKQAHHSNVPGSVFKVCMKQKKKEFKAG

SEQ ID NO: 212 - skipped

SEQ ID NO: 213 - protein, 42 aa, Artificial Sequence
  Synthetic Polypeptide
  DISULFID (14)..(31)
  MOD_RES (30)..(30): Xaa = 2-aminoisobutyric acid
  MOD_RES (42)..(42): C-terminal amidation
SDPTSQFRKAIDDCQKQAHHSNVPGSVFKXCMKQKKKEFKAG

SEQ ID NO: 214 - protein, 41 aa, Artificial Sequence
  Synthetic Polypeptide
  DISULFID (1)..(5)
  DISULFID (14)..(31)
  MOD_RES (41)..(41): C-terminal amidation
CDATCQFRKAIDDCQKQAHHSNVPGSVFKACMKQKKKEFKA

SEQ ID NO: 215 - protein, 42 aa, Artificial Sequence
  Synthetic Polypeptide
  DISULFID (1)..(5)
  DISULFID (14)..(31)
  MOD_RES (30)..(30): Xaa = 2-aminoisobutyric acid
  MOD_RES (42)..(42): C-terminal amidation
CDATCQFRKAIDECQKQAHHSNVPGSVFKXCMKQKKKEFKAG

SEQ ID NO: 216 - protein, 41 aa, Artificial Sequence
  Synthetic Polypeptide
  DISULFID (1)..(5)
  DISULFID (14)..(30)
  MOD_RES (29)..(29): Xaa = 2-aminoisobutyric acid
  MOD_RES (41)..(41): C-terminal amidation
CDATCQFRKAIDDCQKQAHHSNVPGSFKXCMKQKKKEFKAG

SEQ ID NO: 217 - protein, 35 aa, Artificial Sequence
  Synthetic Polypeptide
  DISULFID (1)..(5)
  DISULFID (14)..(26)
  MOD_RES (25)..(25): Xaa = 2-aminoisobutyric acid
  MOD_RES (27)..(27): Xaa = norleucine
  MOD_RES (35)..(35): C-terminal amidation
CDATCQFRKAIDDCQKQAHHSSFKXCXKQKKKEFK

SEQ ID NO: 218 - protein, 36 aa, Artificial Sequence
  Synthetic Polypeptide
  DISULFID (1)..(5)
  DISULFID (14)..(27)
  MOD_RES (26)..(26): Xaa = 2-aminoisobutyric acid
  MOD_RES (28)..(28): Xaa = norleucine
  MOD_RES (36)..(36): C-terminal amidation
CDATCQFRKAIDDCDKQAHHSSVFKXCXKQKKKEFK

SEQ ID NO: 219 - protein, 35 aa, Artificial Sequence
  Synthetic Polypeptide
  DISULFID (1)..(5)
  DISULFID (14)..(26)
  MOD_RES (27)..(27): Xaa = norleucine
  MOD_RES (35)..(35): C-terminal amidation
CDATCQFRKAIDDCDKQAHHSSFKECXKQKKKEFK

SEQ ID NO: 220 - protein, 36 aa, Artificial Sequence
  Synthetic Polypeptide
  DISULFID (1)..(5)
  DISULFID (14)..(27)
  MOD_RES (28)..(28): Xaa = norleucine
  MOD_RES (36)..(36): C-terminal amidation
CDATCQFRKAIDDCDKQAHHSNSFKECXKQKKKEFK

SEQ ID NO: 221 - protein, 36 aa, Artificial Sequence
  Synthetic Polypeptide
  DISULFID (1)..(5)
  DISULFID (14)..(27)
  MOD_RES (28)..(28): Xaa = norleucine
  MOD_RES (36)..(36): C-terminal amidation
CDATCQFRKAIDDCDKQAHHSSVFKECXKQKKKEFK

SEQ ID NO: 222 - protein, 36 aa, Artificial Sequence
  Synthetic Polypeptide
  DISULFID (1)..(5)
  DISULFID (14)..(27)
  MOD_RES (36)..(36): C-terminal amidation
CDATCQFRKAIDDCDKQAHHSNSFKECMKQKKKEFK

SEQ ID NO: 223 - protein, 36 aa, Artificial Sequence
  Synthetic Polypeptide
  DISULFID (1)..(5)
  DISULFID (14)..(27)
  MOD_RES (36)..(36): C-terminal amidation
CDATCQFRKAIDDCDKQAHHSSVFKECMKQKKKEFK

SEQ ID NO: 224 - protein, 36 aa, Artificial Sequence
  Synthetic Polypeptide
  DISULFID (1)..(5)
  DISULFID (14)..(27)
  MOD_RES (36)..(36): C-terminal amidation
CDATCQFRKAIDDCQKQAHHSNSFKECMKQKKKEFK

SEQ ID NO: 225 - protein, 36 aa, Artificial Sequence
  Synthetic Polypeptide
  DISULFID (1)..(5)
  DISULFID (14)..(27)
  MOD_RES (36)..(36): C-terminal amidation
CDATCQFRKAIDDCQKQAHHSSVFKECMKQKKKEFK

SEQ ID NO: 226 - protein, 42 aa, Artificial Sequence
  Synthetic Polypeptide
  DISULFID (1)..(5)
  DISULFID (14)..(31)
  MOD_RES (42)..(42): C-terminal amidation
CDATCQFRKAIDDCQKQAHHSNVPGSVFKLCMKQKKKEFKAG

SEQ ID NO: 227 - protein, 42 aa, Artificial Sequence
  Synthetic Polypeptide
  DISULFID (1)..(5)
  DISULFID (14)..(31)
  MOD_RES (30)..(30): Xaa = 2-aminoisobutyric acid
  MOD_RES (42)..(42): C-terminal amidation
CDATCQFRKAIDDCQKQAHHSNGPAAVFKXCMKQKKKEFKAG

SEQ ID NO: 228 - protein, 42 aa, Artificial Sequence; identical to SEQ ID NO: 206
  Synthetic Polypeptide
  DISULFID (1)..(5)
  DISULFID (14)..(31)
  MOD_RES (30)..(30): Xaa = 2-aminoisobutyric acid
  MOD_RES (42)..(42): C-terminal amidation

SEQ ID NO: 229 - protein, 42 aa, Artificial Sequence
  Synthetic Polypeptide
  DISULFID (1)..(5)
  DISULFID (14)..(31)
  MOD_RES (30)..(30): Xaa = 2-aminoisobutyric acid
  MOD_RES (42)..(42): C-terminal amidation
CDATCQFRKAIDDCDRQAHHSNVPGSVFKXCMKQKKKEFKAG

SEQ ID NO: 230 - protein, 42 aa, Artificial Sequence
  Synthetic Polypeptide
  DISULFID (1)..(5)
  DISULFID (14)..(31)
  MOD_RES (30)..(30): Xaa = D-alanine
  MOD_RES (42)..(42): C-terminal amidation
CDATCQFRKAIDDCQKQAHHSNVPGSVFKXCMKQKKKEFKAG

SEQ ID NO: 231 - protein, 42 aa, Artificial Sequence
  Synthetic Polypeptide
  DISULFID (1)..(5)
  DISULFID (14)..(31)
  MOD_RES (30)..(30): Xaa = 2-aminoisobutyric acid
  MOD_RES (42)..(42): C-terminal amidation
CDATCQFRKAIDDCQKQAHHSNVPGSVFKXCMKQKKKEWKAG

SEQ ID NO: 232 - protein, 15 aa, Artificial Sequence
  Synthetic Polypeptide
  MOD_RES (3)..(3): Xaa = 2-aminoisobutyric acid
  MOD_RES (15)..(15): C-terminal amidation
FKXCMKQKKKEFKAG

SEQ ID NO: 233 - protein, 42 aa, Artificial Sequence; identical to SEQ ID NO: 190
  Synthetic Polypeptide
  DISULFID (1)..(5)
  DISULFID (14)..(31)
  MOD_RES (42)..(42): C-terminal amidation

SEQ ID NO: 234 - protein, 41 aa, Artificial Sequence
  Synthetic Polypeptide
  DISULFID (1)..(5)
  DISULFID (14)..(30)
  MOD_RES (29)..(29): Xaa = 2-aminoisobutyric acid
  MOD_RES (41)..(41): C-terminal amidation
CDATCQFRKAIDDCDKQAHHSNVPGSFKXCMKQKKKEFKAG

SEQ ID NO: 235 - protein, 42 aa, Artificial Sequence
  Synthetic Polypeptide
  DISULFID (1)..(5)
  DISULFID (14)..(31)
  MOD_RES (30)..(30): Xaa = 2-aminoisobutyric acid
  MOD_RES (42)..(42): C-terminal amidation
CDATCQFRKAIDDCQKQAYHSNVPGSVFKXCMKQKKKEFKAG

SEQ ID NO: 236 - protein, 42 aa, Artificial Sequence
  Synthetic Polypeptide
  DISULFID (1)..(5)
  MOD_RES (1)..(1): Xaa = N-terminal acetylation
  DISULFID (14)..(31)
  MOD_RES (30)..(30): Xaa = 2-aminoisobutyric acid
  MOD_RES (42)..(42): C-terminal amidation
CDATCQFRKAIDDCDKQAHHSNVPGSVFKXCMKQKKKEFKAG

SEQ ID NO: 237 - protein, 41 aa, Artificial Sequence
  Synthetic Polypeptide
  DISULFID (1)..(5)
  DISULFID (14)..(30)
  MOD_RES (29)..(29): Xaa = 2-aminoisobutyric acid
  MOD_RES (41)..(41): C-terminal amidation
CDATCQFRKAIDDCQKQAHHSNVPGVFKXCMKQKKKEFKAG

SEQ ID NO: 238 - protein, 41 aa, Artificial Sequence
  Synthetic Polypeptide
  DISULFID (1)..(5)
  DISULFID (14)..(30)
  MOD_RES (29)..(29): Xaa = 2-aminoisobutyric acid
  MOD_RES (41)..(41): C-terminal amidation
CDATCQFRKAIDDCDKQAHHSNVPGVFKXCMKQKKKEFKAG

SEQ ID NO: 239 - protein, 41 aa, Artificial Sequence; identical to SEQ ID NO: 234
  Synthetic Polypeptide
  DISULFID (1)..(5)
  MOD_RES (1)..(1): Xaa = N-terminal acetylation
  DISULFID (14)..(30)
  MOD_RES (29)..(29): Xaa = 2-aminoisobutyric acid
  MOD_RES (41)..(41): C-terminal amidation

SEQ ID NO: 240 - protein, 35 aa, Artificial Sequence
  Synthetic Polypeptide
  DISULFID (1)..(5)
  DISULFID (14)..(26)
  MOD_RES (25)..(25): Xaa = 2-aminoisobutyric acid
  MOD_RES (35)..(35): C-terminal amidation
CDATCQFRKAIDDCDKQAHHSSFKXCMKQKKKEFK

SEQ ID NO: 241 - protein, 36 aa, Artificial Sequence
  Synthetic Polypeptide
  DISULFID (1)..(5)
  DISULFID (14)..(27)
  MOD_RES (26)..(26): Xaa = 2-aminoisobutyric acid
  MOD_RES (28)..(28): Xaa = norleucine
  MOD_RES (36)..(36): C-terminal amidation
CDATCQFRKAIDDCQKQAHHSNSFKXCXKQKKKEFK

SEQ ID NO: 242 - protein, 36 aa, Artificial Sequence
  Synthetic Polypeptide
  DISULFID (1)..(5)
  DISULFID (14)..(27)
  MOD_RES (26)..(26): Xaa = 2-aminoisobutyric acid
  MOD_RES (28)..(28): Xaa = norleucine
  MOD_RES (36)..(36): C-terminal amidation
CDATCQFRKAIDDCQKQAHHSSVFKXCXKQKKKEFK

SEQ ID NO: 243 - protein, 35 aa, Artificial Sequence
  Synthetic Polypeptide
  DISULFID (1)..(5)
  DISULFID (14)..(26)
  MOD_RES (25)..(25): Xaa = 2-aminoisobutyric acid
  MOD_RES (35)..(35): C-terminal amidation
CDATCQFRKAIDDCQKQAHHSSFKXCMKQKKKEFK

SEQ ID NO: 244 - protein, 36 aa, Artificial Sequence
  Synthetic Polypeptide
  DISULFID (1)..(5)
  DISULFID (14)..(27)
  MOD_RES (26)..(26): Xaa = 2-aminoisobutyric acid
  MOD_RES (36)..(36): C-terminal amidation
CDATCQFRKAIDDCDKQAHHSNSFKXCMKQKKKEFK

SEQ ID NO: 245 - protein, 36 aa, Artificial Sequence
  Synthetic Polypeptide
  DISULFID (1)..(5)
  DISULFID (14)..(27)
  MOD_RES (26)..(26): Xaa = 2-aminoisobutyric acid
  MOD_RES (36)..(36): C-terminal amidation
CDATCQFRKAIDDCDKQAHHSSVFKXCMKQKKKEFK

SEQ ID NO: 246 - protein, 37 aa, Artificial Sequence
  Synthetic Polypeptide
  DISULFID (1)..(5)
  DISULFID (14)..(28)
  MOD_RES (27)..(27): Xaa = 2-aminoisobutyric acid
  MOD_RES (29)..(29): Xaa = norleucine
  MOD_RES (37)..(37): C-terminal amidation
CDATCQFRKAIDDCQKQAHHSNSVFKXCXKQKKKEFK

SEQ ID NO: 247 - protein, 36 aa, Artificial Sequence
  Synthetic Polypeptide
  DISULFID (1)..(5)
  DISULFID (14)..(27)
  MOD_RES (26)..(26): Xaa = 2-aminoisobutyric acid
  MOD_RES (36)..(36): C-terminal amidation
CDATCQFRKAIDDCQKQAHHSNSFKXCMKQKKKEFK

SEQ ID NO: 248 - protein, 41 aa, Artificial Sequence
  Synthetic Polypeptide
  DISULFID (1)..(5)
  DISULFID (14)..(30)
  MOD_RES (29)..(29): Xaa = 2-aminoisobutyric acid
  MOD_RES (31)..(31): Xaa = norleucine
  MOD_RES (41)..(41): C-terminal amidation
CDATCQFRKAIDDCDKQAHHSNVPSVFKXCXKQKKKEFKAG

SEQ ID NO: 249 - protein, 41 aa, Artificial Sequence
  Synthetic Polypeptide
  DISULFID (1)..(5)
  MOD_RES (1)..(1): Xaa = N-terminal acetylation
  DISULFID (14)..(31)
  MOD_RES (30)..(30): Xaa = 2-aminoisobutyric acid
  MOD_RES (41)..(41): C-terminal amidation
CDATCQFRKAIDDCQKQAHHSNVPGSVFKXCMKQKKKEFKA

SEQ ID NO: 250 - protein, 41 aa, Artificial Sequence; identical to SEQ ID NO: 249
  Synthetic Polypeptide
  DISULFID (1)..(5)
  DISULFID (14)..(31)
  MOD_RES (30)..(30): Xaa = 2-aminoisobutyric acid
  MOD_RES (41)..(41): C-terminal amidation

SEQ ID NO: 251 - protein, 41 aa, Artificial Sequence
  Synthetic Polypeptide
  DISULFID (1)..(5)
  DISULFID (14)..(30)
  MOD_RES (29)..(29): Xaa = 2-aminoisobutyric acid
  MOD_RES (31)..(31): Xaa = norleucine
  MOD_RES (41)..(41): C-terminal amidation
CDATCQFRKAIDDCDKQAYHSNVPSVFKXCXKQKKKEFKAG

SEQ ID NO: 252 - protein, 41 aa, Artificial Sequence
  Synthetic Polypeptide
  DISULFID (1)..(5)
  DISULFID (14)..(30)
  MOD_RES (29)..(29): Xaa = 2-aminoisobutyric acid
  MOD_RES (31)..(31): Xaa = norleucine
  MOD_RES (41)..(41): C-terminal amidation
CDATCQFRKAIDDCDKQAHHSNVPGSFKXCXKQKKKEFKAG

SEQ ID NO: 253 - protein, 42 aa, Artificial Sequence; identical to SEQ ID NO: 230
  Synthetic Polypeptide
  MOD_RES (1)..(1): Xaa = N-terminal acetylation
  DISULFID (1)..(5)
  DISULFID (14)..(31)
  MOD_RES (30)..(30): Xaa = 2-aminoisobutyric acid
  MOD_RES (42)..(42): C-terminal amidation

SEQ ID NO: 254 - protein, 42 aa, Artificial Sequence; identical to SEQ ID NO: 236
  Synthetic Polypeptide
  DISULFID (1)..(5)
  DISULFID (14)..(31)
  MOD_RES (30)..(30): Xaa = 2-aminoisobutyric acid
  MOD_RES (42)..(42): C-terminal amidation

SEQ ID NO: 255 - protein, 42 aa, Artificial Sequence
  Synthetic Polypeptide
  DISULFID (1)..(5)
  DISULFID (14)..(31)
  MOD_RES (30)..(30): Xaa = 2-aminoisobutyric acid
  MOD_RES (32)..(32): Xaa = norleucine
  MOD_RES (42)..(42): C-terminal amidation
CDATCQFRKAIDDCDKQAHHSNVPGSVFKXCXKQKKKEFKAG

SEQ ID NO: 256 - protein, 37 aa, Artificial Sequence
  Synthetic Polypeptide
  DISULFID (1)..(5)
  DISULFID (14)..(28)
  MOD_RES (27)..(27): Xaa = 2-aminoisobutyric acid
  MOD_RES (37)..(37): C-terminal amidation
CDATCQFRKAIDDCQKQAHHSNSVFKXCMKQKKKEFK

SEQ ID NO: 257 - protein, 39 aa, Artificial Sequence
  Synthetic Polypeptide
  DISULFID (1)..(5)
  DISULFID (14)..(30)
  MOD_RES (29)..(29): Xaa = 2-aminoisobutyric acid
  MOD_RES (31)..(31): Xaa = norleucine
  MOD_RES (39)..(39): C-terminal amidation
CDATCQFRKAIDDCDKQAHHSNVPGSFKXCXKQKKKEFK

SEQ ID NO: 258 - protein, 40 aa, Artificial Sequence
  Synthetic Polypeptide
  DISULFID (1)..(5)
  DISULFID (14)..(31)
  MOD_RES (30)..(30): Xaa = 2-aminoisobutyric acid
  MOD_RES (32)..(32): Xaa = norleucine
  MOD_RES (40)..(40): C-terminal amidation
CDATCQFRKAIDDCDKQAHHSNVPGNSFKXCXKQKKKEFK

SEQ ID NO: 259 - protein, 40 aa, Artificial Sequence
  Synthetic Polypeptide
  DISULFID (1)..(5)
  DISULFID (14)..(31)
  MOD_RES (30)..(30): Xaa = 2-aminoisobutyric acid
  MOD_RES (32)..(32): Xaa = norleucine
  MOD_RES (40)..(40): C-terminal amidation
CDATCQFRKAIDDCDKQAHHSNVPGSVFKXCXKQKKKEFK

SEQ ID NO: 260 - protein, 40 aa, Artificial Sequence
  Synthetic Polypeptide
  DISULFID (1)..(5)
  MOD_RES (1)..(1): Xaa = N-terminal acetylation
  DISULFID (14)..(31)
  MOD_RES (30)..(30): Xaa = 2-aminoisobutyric acid
  MOD_RES (32)..(32): Xaa = norleucine
  MOD_RES (40)..(40): C-terminal amidation
CDATCQFRKAIDDCQKQAHHSNVPGSVFKXCXKQKKKEFK

SEQ ID NO: 261 - protein, 41 aa, Artificial Sequence
  Synthetic Polypeptide
  DISULFID (1)..(5)
  DISULFID (14)..(32)
  MOD_RES (31)..(31): Xaa = 2-aminoisobutyric acid
  MOD_RES (33)..(33): Xaa = norleucine
  MOD_RES (41)..(41): C-terminal amidation
CDATCQFRKAIDDCDKQAHHSNVPGNSVFKXCXKQKKKEFK

SEQ ID NO: 262 - protein, 41 aa, Artificial Sequence
  Synthetic Polypeptide
  DISULFID (1)..(5)
  DISULFID (14)..(30)
  MOD_RES (29)..(29): Xaa = 2-aminoisobutyric acid
  MOD_RES (41)..(41): C-terminal amidation
CDATCQFRKAIDDCQKQAHHSNVGSVFKXCMKQKKKEFKAG

SEQ ID NO: 263 - protein, 42 aa, Artificial Sequence
  Synthetic Polypeptide
  DISULFID (1)..(5)
  DISULFID (14)..(31)
  MOD_RES (30)..(30): Xaa = 2-aminoisobutyric acid
  MOD_RES (32)..(32): Xaa = norleucine
  MOD_RES (42)..(42): C-terminal amidation
CDATCQFRKAIDDCQKQAHHSNVPGSVFKXCXKQKKKEFKAG

SEQ ID NO: 264 - protein, 40 aa, Artificial Sequence; identical to SEQ ID NO: 260
  Synthetic Polypeptide
  DISULFID (1)..(5)
  DISULFID (14)..(31)
  MOD_RES (30)..(30): Xaa = 2-aminoisobutyric acid
  MOD_RES (32)..(32): Xaa = norleucine
  MOD_RES (40)..(40): C-terminal amidation

SEQ ID NO: 265 - protein, 40 aa, Artificial Sequence
  Synthetic Polypeptide
  DISULFID (1)..(4)
  DISULFID (13)..(31)
  MOD_RES (39)..(39): Xaa = alpha-methyl-phenylalanine
  MOD_RES (40)..(40): C-terminal amidation
CDACQFRKAIDDCQKQAHHSNVPGNSVFKECMKQKKKEXK

SEQ ID NO: 266 - protein, 41 aa, Artificial Sequence
  Synthetic Polypeptide
  DISULFID (1)..(5)
  DISULFID (14)..(32)
  MOD_RES (33)..(33): Xaa = norleucine
  MOD_RES (41)..(41): C-terminal amidation
CDATCQFRKAIDDCDKQAHHSNVPGNSVFKECXKQKKKEFK

SEQ ID NO: 267 - protein, 40 aa, Artificial Sequence
  Synthetic Polypeptide
  DISULFID (1)..(5)
  DISULFID (14)..(31)
  MOD_RES (30)..(30): Xaa = 2-aminoisobutyric acid
  MOD_RES (32)..(32): Xaa = norleucine
  MOD_RES (40)..(40): C-terminal amidation
CDATCQFRKAIDDCQKQAHHSNVPGNSFKXCXKQKKKEFK

SEQ ID NO: 268 - protein, 41 aa, Artificial Sequence
  Synthetic Polypeptide
  DISULFID (1)..(5)
  DISULFID (14)..(32)
  MOD_RES (31)..(31): Xaa = 2-aminoisobutyric acid
  MOD_RES (33)..(33): Xaa = norleucine
  MOD_RES (41)..(41): C-terminal amidation
CDATCQFRKAIDDCQKQAHHSNVPGNSVFKXCXKQKKKEFK

SEQ ID NO: 269 - protein, 40 aa, Artificial Sequence
  Synthetic Polypeptide
  DISULFID (1)..(5)
  DISULFID (14)..(31)
  MOD_RES (32)..(32): Xaa = norleucine
  MOD_RES (40)..(40): C-terminal amidation
CDATCQFRKAIDDCQKQAHHSNVPGSVFKECXKQKKKEFK

SEQ ID NO: 270 - protein, 40 aa, Artificial Sequence
  Synthetic Polypeptide
  DISULFID (1)..(5)
  DISULFID (14)..(31)
  MOD_RES (30)..(30): Xaa = 2-aminoisobutyric acid
  MOD_RES (40)..(40): C-terminal amidation
CDATCQFRKAIDDCDKQAHHSNVPGNSFKXCMKQKKKEFK

SEQ ID NO: 271 - protein, 40 aa, Artificial Sequence
  Synthetic Polypeptide
  DISULFID (1)..(5)
  DISULFID (14)..(31)
  MOD_RES (30)..(30): Xaa = 2-aminoisobutyric acid
  MOD_RES (40)..(40): C-terminal amidation
CDATCQFRKAIDDCDKQAHHSNVPGSVFKXCMKQKKKEFK

SEQ ID NO: 272 - protein, 42 aa, Artificial Sequence
  Synthetic Polypeptide
  DISULFID (1)..(5)
  DISULFID (14)..(32)
CDATCQFRKAIDDCQKQAHHSNVPGNSVFKECMKQKKKEFKA

SEQ ID NO: 273 - protein, 43 aa, Artificial Sequence
  Synthetic Polypeptide
  DISULFID (1)..(5)
  DISULFID (14)..(32)
CDATCQFRKAIDDCQKQAHHSNVPGNSVFKECMKQKKKEFKAG

SEQ ID NO: 274 - protein, 35 aa, Artificial Sequence
  Synthetic Polypeptide
  DISULFID (1)..(5)
  DISULFID (14)..(26)
  MOD_RES (25)..(25): Xaa = 2-aminoisobutyric acid
  MOD_RES (27)..(27): Xaa = norleucine
  MOD_RES (35)..(35): C-terminal amidation
CDATCQFRKAIDDCDKQAHHSSFKXCXKQKKKEFK

SEQ ID NO: 275 - protein, 40 aa, Artificial Sequence
  Synthetic Polypeptide
  DISULFID (1)..(5)
  DISULFID (14)..(31)
  MOD_RES (40)..(40): C-terminal amidation
CDATCQFRKAIDDCQKQAHHSNVGNSVFKECMKQKKKEFK

SEQ ID NO: 276 - protein, 41 aa, Artificial Sequence
  Synthetic Polypeptide
  DISULFID (1)..(5)
  DISULFID (14)..(32)
  MOD_RES (41)..(41): C-terminal amidation
CDATCQFRKAIDDCQKQAHHSNVPGNSVFKECMKQKKQEFK

SEQ ID NO: 277 - protein, 41 aa, Artificial Sequence
  Synthetic Polypeptide
  DISULFID (1)..(5)
  DISULFID (14)..(32)
  MOD_RES (38)..(38): Xaa = ornithine
  MOD_RES (41)..(41): C-terminal amidation
CDATCQFRKAIDDCQKQAHHSNVPGNSVFKECMKQKKXEFK

SEQ ID NO: 278 - protein, 41 aa, Artificial Sequence; identical to SEQ ID NO: 277
  Synthetic Polypeptide
  DISULFID (1)..(5)
  DISULFID (14)..(32)
  MOD_RES (38)..(38): Xaa = D-Lysine
  MOD_RES (41)..(41): C-terminal amidation

SEQ ID NO: 279 - protein, 41 aa, Artificial Sequence
  Synthetic Polypeptide
  DISULFID (1)..(5)
  DISULFID (14)..(32)
  MOD_RES (41)..(41): C-terminal amidation
CDATCQFRKAIDDCQKQAHHSNVPGNSVFKECMKQKKAEFK

SEQ ID NO: 280 - protein, 41 aa, Artificial Sequence
  Synthetic Polypeptide
  DISULFID (1)..(5)
  DISULFID (14)..(32)
  MOD_RES (41)..(41): C-terminal amidation
CDATCQFRKAIDDCQKQAHHSNVPGNSVFKECMKQKKGEFK

SEQ ID NO: 281 - protein, 41 aa, Artificial Sequence
  Synthetic Polypeptide
  DISULFID (1)..(5)
  DISULFID (14)..(32)
  MOD_RES (36)..(36): Xaa = D-lysine
  MOD_RES (41)..(41): C-terminal amidation
CDATCQFRKAIDDCQKQAHHSNVPGNSVFKECMKQXKKEFK

SEQ ID NO: 282 - protein, 41 aa, Artificial Sequence
  Synthetic Polypeptide
  DISULFID (1)..(5)
  DISULFID (14)..(32)
  MOD_RES (40)..(40): Xaa = homophenylalanine
  MOD_RES (41)..(41): C-terminal amidation
CDATCQFRKAIDDCQKQAHHSNVPGNSVFKECMKQKKKEXK

SEQ ID NO: 283 - protein, 42 aa, Artificial Sequence; identical to SEQ ID NO: 230
  Synthetic Polypeptide
  DISULFID (1)..(5)
  DISULFID (14)..(31)
  MOD_RES (30)..(30): Xaa = 2-aminoisobutyric acid
  MOD_RES (42)..(42): C-terminal amidation

SEQ ID NO: 284 - protein, 41 aa, Artificial Sequence
  Synthetic Polypeptide
  DISULFID (1)..(5)
  DISULFID (14)..(32)
  MOD_RES (41)..(41): C-terminal amidation
CDATCQFRKAIDDCQKQAHHSNVPGNSVFKECMKQKQKEFK

SEQ ID NO: 285 - protein, 41 aa, Artificial Sequence
  Synthetic Polypeptide
  DISULFID (1)..(5)
  DISULFID (14)..(32)
  MOD_RES (41)..(41): C-terminal amidation
CDATCQFRKAIDDCQKQAHHSNVPGNSVFKECMKQGKKEFK

SEQ ID NO: 286 - protein, 41 aa, Artificial Sequence
  Synthetic Polypeptide
  DISULFID (1)..(5)
  DISULFID (14)..(32)
  MOD_RES (17)..(17): Xaa = 2-aminoisobutyric acid
  MOD_RES (41)..(41): C-terminal amidation
CDATCQFRKAIDDCQKXAHHSNVPGNSVFKECMKQKKKEFK

SEQ ID NO: 287 - protein, 41 aa, Artificial Sequence
  Synthetic Polypeptide
  DISULFID (1)..(5)
  DISULFID (14)..(32)
  MOD_RES (41)..(41): C-terminal amidation
CDATCQFRKAIDDCQKQAHHSNVPGNSVFKECMKQKKKAFK

SEQ ID NO: 288 - protein, 41 aa, Artificial Sequence
  Synthetic Polypeptide
  DISULFID (1)..(5)
  DISULFID (14)..(32)
  MOD_RES (41)..(41): C-terminal amidation
CDATCQFRKAIDDCQRQAHHSNVPGNSVFKECMKQKKKEFK

SEQ ID NO: 289 - protein, 41 aa, Artificial Sequence
  Synthetic Polypeptide
  DISULFID (1)..(5)
  DISULFID (14)..(32)
  MOD_RES (20)..(20): Xaa = 2-aminoisobutyric acid
  MOD_RES (41)..(41): C-terminal amidation
CDATCQFRKAIDDCQKQAHXSNVPGNSVFKECMKQKKKEFK

SEQ ID NO: 290 - protein, 44 aa, Artificial Sequence
  Synthetic Polypeptide
  DISULFID (1)..(5)
  MOD_RES (1)..(1): Xaa = N-terminal acetylation
  DISULFID (14)..(32)
CDATCQFRKAIDDCQKQAHHSNVPGNSVFKECMKQKKKEFKAGK

SEQ ID NO: 291 - protein, 41 aa, Artificial Sequence; identical to SEQ ID NO: 277
  Synthetic Polypeptide
  DISULFID (1)..(5)
  DISULFID (14)..(32)
  MOD_RES (38)..(38): Xaa = N -methyllysine
  MOD_RES (41)..(41): C-terminal amidation

SEQ ID NO: 292 - protein, 41 aa, Artificial Sequence
  Synthetic Polypeptide
  DISULFID (1)..(5)
  DISULFID (14)..(32)
  MOD_RES (41)..(41): Xaa = C-terminal amidation
  MOD_RES (41)..(41): Xaa = N -methyllysine
CDATCQFRKAIDDCQKQAHHSNVPGNSVFKECMKQKKKEFX

SEQ ID NO: 293 - protein, 40 aa, Artificial Sequence
  Synthetic Polypeptide
  DISULFID (1)..(5)
  DISULFID (14)..(31)
  MOD_RES (40)..(40): C-terminal amidation
CDATCQFRKAIDDCQKQAHHSNVPGSVFKECMKQKKKEFK

SEQ ID NO: 294 - protein, 44 aa, Artificial Sequence; identical to SEQ ID NO: 290
  Synthetic Polypeptide
  DISULFID (1)..(5)
  DISULFID (14)..(32)
  MOD_RES (44)..(44): C-terminal amidation

SEQ ID NO: 295 - protein, 41 aa, Artificial Sequence
  Synthetic Polypeptide
  DISULFID (1)..(5)
  DISULFID (14)..(32)
  MOD_RES (41)..(41): C-terminal amidation
CDATCQFRKAIDDCDKQAHHSNVPGNSVFKECMKQKKKEFK

SEQ ID NO: 296 - protein, 41 aa, Artificial Sequence
  Synthetic Polypeptide
  DISULFID (1)..(5)
  DISULFID (14)..(32)
  MOD_RES (31)..(31): Xaa = 2-aminoisobutyric acid
  MOD_RES (41)..(41): C-terminal amidation
CDATCQFRKAIDDCQKQAHHSNVPGNSVFKXCMKQKKKEFK

SEQ ID NO: 297 - protein, 41 aa, Artificial Sequence; identical to SEQ ID NO: 282
  Synthetic Polypeptide
  DISULFID (1)..(5)
  DISULFID (14)..(32)
  MOD_RES (40)..(40): Xaa = alpha-methyl-phenylalanine
  MOD_RES (41)..(41): C-terminal amidation

SEQ ID NO: 298 - protein, 41 aa, Artificial Sequence
  Synthetic Polypeptide
  DISULFID (1)..(5)
  DISULFID (14)..(32)
  MOD_RES (33)..(33): Xaa = norleucine
  MOD_RES (41)..(41): C-terminal amidation
CDATCQFRKAIDDCQKQAHHSNVPGNSVFKECXKQKKKEFK

SEQ ID NO: 299 - protein, 41 aa, Artificial Sequence; identical to SEQ ID NO: 281
  Synthetic Polypeptide
  DISULFID (1)..(5)
  DISULFID (14)..(32)
  MOD_RES (36)..(36): Xaa = ornithine
  MOD_RES (41)..(41): C-terminal amidation

SEQ ID NO: 300 - protein, 44 aa, Artificial Sequence
  Synthetic Polypeptide
  DISULFID (1)..(5)
  DISULFID (14)..(32)
CDATCQFRKAIDDCQKQAHHSNVPGNSVFKECMKQKKKEFKAGH

SEQ ID NO: 301 - protein, 41 aa, Artificial Sequence
  Synthetic Polypeptide
  DISULFID (1)..(5)
  DISULFID (14)..(32)
  MOD_RES (41)..(41): C-terminal amidation
CDATCQFRKAIDDCQKQAHHSNVPGNSVFKECMKQKKKEWK

SEQ ID NO: 302 - protein, 41 aa, Artificial Sequence
  Synthetic Polypeptide
  DISULFID (1)..(5)
  DISULFID (14)..(32)
  MOD_RES (41)..(41): C-terminal amidation
CDATCQFRKAIDDCQKQAHHSNVPGNSVFKECMKQKKKEFH

SEQ ID NO: 303 - protein, 41 aa, Artificial Sequence
  Synthetic Polypeptide
  DISULFID (1)..(5)
  DISULFID (14)..(32)
  MOD_RES (41)..(41): C-terminal amidation
CDATCQFRKAIDDCQKQAHHSNVPGNSVFKECMKQKKKEFQ

SEQ ID NO: 304 - protein, 41 aa, Artificial Sequence; identical to SEQ ID NO: 292
  Synthetic Polypeptide
  DISULFID (1)..(5)
  DISULFID (14)..(32)
  MOD_RES (41)..(41): Xaa = C-terminal amidation
  MOD_RES (41)..(41): Xaa = D-lysine

SEQ ID NO: 305 - skipped

SEQ ID NO: 306 - protein, 41 aa, Artificial Sequence
  Synthetic Polypeptide
  DISULFID (1)..(5)
  DISULFID (14)..(32)
  MOD_RES (41)..(41): C-terminal amidation
CDATCQFRKAIDDCQKQAYHSNVPGNSVFKECMKQKKKEFK

SEQ ID NO: 307 - protein, 41 aa, Artificial Sequence
  Synthetic Polypeptide
  DISULFID (1)..(5)
  DISULFID (14)..(32)
  MOD_RES (41)..(41): C-terminal amidation
CDATCQFRKAIDDCQKQAHHSNVPGNSVFKECMKQQKKEFK

SEQ ID NO: 308 - protein, 41 aa, Artificial Sequence
  Synthetic Polypeptide
  DISULFID (1)..(5)
  DISULFID (14)..(32)
  MOD_RES (41)..(41): C-terminal amidation
CDATCQFRKAIDDCQKQAHHSNVPGNSVFKECMKQAKKEFK

SEQ ID NO: 309 - protein, 41 aa, Artificial Sequence; identical to SEQ ID NO: 282
  Synthetic Polypeptide
  DISULFID (1)..(5)
  DISULFID (14)..(32)
  MOD_RES (40)..(40): Xaa = D-phenylalanine
  MOD_RES (41)..(41): C-terminal amidation

SEQ ID NO: 310 - protein, 41 aa, Artificial Sequence
  Synthetic Polypeptide
  DISULFID (1)..(5)
  DISULFID (14)..(32)
  MOD_RES (41)..(41): C-terminal amidation
CDATCQFRKAIDDCQKQAHHSNVPGNSVFKECMKQKKKEFE

SEQ ID NO: 311 - protein, 40 aa, Artificial Sequence
  Synthetic Polypeptide
  DISULFID (1)..(5)
  DISULFID (14)..(31)
  MOD_RES (40)..(40): C-terminal amidation
CDATCQFRKAIDDCQKQAHHSNVPNSVFKECMKQKKKEFK

SEQ ID NO: 312 - protein, 44 aa, Artificial Sequence
  Synthetic Polypeptide
  DISULFID (1)..(5)
  DISULFID (14)..(32)
  MOD_RES (40)..(40): Xaa = homophenylalanine
CDATCQFRKAIDDCQKQAHHSNVPGNSVFKECMKQKKKEXKAGK

SEQ ID NO: 313 - protein, 41 aa, Artificial Sequence
  Synthetic Polypeptide
  DISULFID (1)..(5)
  DISULFID (14)..(32)
CDATCQFRKAIDDCQKQAHHSNVPGNSVFKECMKQKKKEFK

SEQ ID NO: 314 - protein, 44 aa, Artificial Sequence
  Synthetic Polypeptide
  DISULFID (1)..(5)
  DISULFID (14)..(32)
CDATCQFRKAIDDCQKQAHHSNVPGNSVFKECMKQKKKEFKPGK

SEQ ID NO: 315 - protein, 44 aa, Artificial Sequence
  Synthetic Polypeptide
  DISULFID (1)..(5)
  DISULFID (14)..(32)
CDATCQFRKAIDDCQKQAHHSNVPGNSVFKECMKQKKKEWKAGK

SEQ ID NO: 316 - protein, 44 aa, Artificial Sequence
  Synthetic Polypeptide
  DISULFID (1)..(5)
  DISULFID (14)..(32)
CDATCQFRKAIDDCQKQAHHSNVPGNSVFKECMKQKKKEFEAGK

SEQ ID NO: 317 - protein, 44 aa, Artificial Sequence
  Synthetic Polypeptide
  DISULFID (1)..(5)
  DISULFID (14)..(32)
CDATCQFRKAIDDCQKQAHHSNVPGNSVFKECMKQKKKEFQAGK

SEQ ID NO: 318 - protein, 44 aa, Artificial Sequence
  Synthetic Polypeptide
  DISULFID (1)..(5)
  DISULFID (14)..(32)
  MOD_RES (41)..(41): Xaa = D-lysine
CDATCQFRKAIDDCQKQAHHSNVPGNSVFKECMKQKKKEFXAGK

SEQ ID NO: 319 - protein, 44 aa, Artificial Sequence
  Synthetic Polypeptide
  DISULFID (1)..(5)
  DISULFID (14)..(32)
CDATCQFRKAIDDCQKQAHHSNVPGNSVFKECMKQKKKEYKAGK

SEQ ID NO: 320 - protein, 44 aa, Artificial Sequence
  Synthetic Polypeptide
  DISULFID (1)..(5)
  DISULFID (14)..(32)
CDATCQFRKAIDDCQKQAHHSNVPGNSVFKECMKQHKKEFKAGK

SEQ ID NO: 321 - protein, 44 aa, Artificial Sequence
  Synthetic Polypeptide
  DISULFID (1)..(5)
  DISULFID (14)..(32)
CDATCQFRKAIDDCQKQAHHSNVPGNSVFKECMKQQKKEFKAGK

SEQ ID NO: 322 - protein, 44 aa, Artificial Sequence
  Synthetic Polypeptide
  DISULFID (1)..(5)
  DISULFID (14)..(32)
  MOD_RES (36)..(36): Xaa = D-lysine
CDATCQFRKAIDDCQKQAHHSNVPGNSVFKECMKQXKKEFKAGK

SEQ ID NO: 323 - protein, 44 aa, Artificial Sequence
  Synthetic Polypeptide
  DISULFID (1)..(5)
  DISULFID (14)..(32)
CDATCQFRKAIDDCQKQAHHSNVPGNSVFKECMKNKKKEFKAGK

SEQ ID NO: 324 - protein, 44 aa, Artificial Sequence
  Synthetic Polypeptide
  DISULFID (1)..(5)
  DISULFID (14)..(32)
CDATCQFRKAIDDCQKQAHHSNVPGNSVFKECMKPKKKEFKAGK

SEQ ID NO: 325 - protein, 44 aa, Artificial Sequence
  Synthetic Polypeptide
  DISULFID (1)..(5)
  DISULFID (14)..(32)
CDATCQFRKAIDDCQKQAHHSNVPGNSVFKECMKEKKKEFKAGK

SEQ ID NO: 326 - protein, 44 aa, Artificial Sequence
  Synthetic Polypeptide
  DISULFID (1)..(5)
  DISULFID (14)..(32)
CDATCQFRKAIDDCQKQAHHSNVPGNSVFKECMKQAKKEFKAGK

SEQ ID NO: 327 - protein, 44 aa, Artificial Sequence
  Synthetic Polypeptide
  DISULFID (1)..(5)
  DISULFID (14)..(32)
CDATCQFRKAIDDCQKQAHHSNVPGNSVFKECMKTKKKEFKAGK

SEQ ID NO: 328 - protein, 44 aa, Artificial Sequence; identical to SEQ ID NO: 290
  Synthetic Polypeptide
  DISULFID (1)..(5)
  MOD_RES (1)..(1): Xaa = N-terminal acetylation
  DISULFID (14)..(32)
  MOD_RES (44)..(44): C-terminal amidation

SEQ ID NO: 329 - protein, 44 aa, Artificial Sequence
  Synthetic Polypeptide
  DISULFID (1)..(5)
  DISULFID (14)..(32)
CDATCQFRKAIDDCQKQAHHSNVPGNSVFEKCMKQKKKEFKAGK

SEQ ID NO: 330 - protein, 44 aa, Artificial Sequence
  Synthetic Polypeptide
  DISULFID (1)..(5)
  DISULFID (14)..(32)
CDATCQFRKAIDDCQKQAHHSNVPGNSVWKECMKQKKKEFKAGK

SEQ ID NO: 331 - protein, 44 aa, Artificial Sequence
  Synthetic Polypeptide
  DISULFID (1)..(5)
  DISULFID (14)..(32)
CDATCQFRKAIDDCQKQAHHSNVPGNSVYKECMKQKKKEFKAGK

SEQ ID NO: 332 - protein, 44 aa, Artificial Sequence
  Synthetic Polypeptide
  DISULFID (1)..(5)
  DISULFID (14)..(32)
CDATCQFRKAIDDCQKQAHHSNVPGQSVFKECMKQKKKEFKAGK

SEQ ID NO: 333 - protein, 44 aa, Artificial Sequence
  Synthetic Polypeptide
  DISULFID (1)..(5)
  DISULFID (14)..(32)
CDATCQFRKAIDDCQKQAHHSHVPGNSVFKECMKQKKKEFKAGK

SEQ ID NO: 334 - protein, 44 aa, Artificial Sequence
  Synthetic Polypeptide
  DISULFID (1)..(5)
  DISULFID (14)..(32)
  MOD_RES (24)..(24): Xaa = pipecolic acid
CDATCQFRKAIDDCQKQAHHSNVXGNSVFKECMKQKKKEFKAGK

SEQ ID NO: 335 - protein, 44 aa, Artificial Sequence
  Synthetic Polypeptide
  DISULFID (1)..(5)
  DISULFID (14)..(32)
CDATCQFRKAIDDCQKQAHHSNVPGNSVFKECMKQKKKEEKAGK

SEQ ID NO: 336 - protein, 44 aa, Artificial Sequence
  Synthetic Polypeptide
  DISULFID (1)..(5)
  DISULFID (14)..(32)
CDATCQFRKAIDDCQKQAHHSNVPGNSVFKECMKQKKEEFKAGK

SEQ ID NO: 337 - protein, 44 aa, Artificial Sequence
  Synthetic Polypeptide
  DISULFID (1)..(5)
  MOD_RES (13)..(13): Xaa = 2-aminoisobutyric acid
  DISULFID (14)..(32)
CDATCQFRKAIDXCQKQAHHSNVPGNSVFKECMKQKKKEFKAGK

SEQ ID NO: 338 - protein, 44 aa, Artificial Sequence
  Synthetic Polypeptide
  DISULFID (1)..(5)
  MOD_RES (11)..(11): Xaa = 2-aminoisobutyric acid
  DISULFID (14)..(32)
CDATCQFRKAXDDCQKQAHHSNVPGNSVFKECMKQKKKEFKAGK

SEQ ID NO: 339 - protein, 44 aa, Artificial Sequence
  Synthetic Polypeptide
  DISULFID (1)..(5)
  DISULFID (14)..(32)
  MOD_RES (44)..(44): Xaa = D-lysine
CDATCQFRKAIDDCQKQAHHSNVPGNSVFKECMKQKKKEFKAGX

SEQ ID NO: 340 - protein, 44 aa, Artificial Sequence
  Synthetic Polypeptide
  DISULFID (1)..(5)
  DISULFID (14)..(32)
CDATCQFRKAIDDCQKQAHHSNVPGNSVFKECMKQEKKEFKAGK

SEQ ID NO: 341 - protein, 44 aa, Artificial Sequence
  Synthetic Polypeptide
  DISULFID (1)..(5)
  DISULFID (14)..(32)
CDATCQFRKAIDDCQKQAHHSNVPGNSVFKECMEQKKKEFKAGK

SEQ ID NO: 342 - protein, 44 aa, Artificial Sequence
  Synthetic Polypeptide
  DISULFID (1)..(5)
  DISULFID (14)..(32)
CDATCQFRKAIDDCQKQAHHSNVPGNSVFKECEKQKKKEFKAGK

SEQ ID NO: 343 - protein, 44 aa, Artificial Sequence
  Synthetic Polypeptide
  DISULFID (1)..(5)
  DISULFID (14)..(32)
CDATCQFRKAIDDCQKQAHHSNVPGNSVFKECMKQKKKEFKAAK

SEQ ID NO: 344 - protein, 44 aa, Artificial Sequence
  Synthetic Polypeptide
  DISULFID (1)..(5)
  DISULFID (14)..(32)
CDATCQFRKAIDDCQKQAHHSNVPGNSVFKECMKQKKKEFAAGK

SEQ ID NO: 345 - protein, 44 aa, Artificial Sequence
  Synthetic Polypeptide
  DISULFID (1)..(5)
  DISULFID (14)..(32)
  MOD_RES (35)..(35): Xaa = 2-aminoisobutyric acid
CDATCQFRKAIDDCQKQAHHSNVPGNSVFKECMKXKKKEFKAGK

SEQ ID NO: 346 - protein, 44 aa, Artificial Sequence
  Synthetic Polypeptide
  DISULFID (1)..(5)
  DISULFID (14)..(32)
CDATCQFRKAIDDCKQQAHHSNVPGNSVFEKCMKQKKKEFKAGK

SEQ ID NO: 347 - protein, 44 aa, Artificial Sequence
  Synthetic Polypeptide
  DISULFID (1)..(5)
  DISULFID (14)..(32)
CDATCQFRKAIDDCQKQAHHSQVPGNSVFKECMKQKKKEFKAGK

SEQ ID NO: 348 - protein, 44 aa, Artificial Sequence
  Synthetic Polypeptide
  DISULFID (1)..(5)
  DISULFID (14)..(32)
  MOD_RES (17)..(17): Xaa = citrulline
CDATCQFRKAIDDCQKXAHHSNVPGNSVFKECMKQKKKEFKAGK

SEQ ID NO: 349 - protein, 44 aa, Artificial Sequence
  Synthetic Polypeptide
  DISULFID (1)..(5)
  DISULFID (14)..(32)
CDATCQFRKAIDDCQKDAHHSNVPGNSVFKECMKQKKKEFKAGK

SEQ ID NO: 350 - protein, 44 aa, Artificial Sequence
  Synthetic Polypeptide
  DISULFID (1)..(5)
  DISULFID (14)..(32)
CDATCQFRKAIDDCQQQAHHSNVPGNSVFKECMKQKKKEFKAGK

SEQ ID NO: 351 - protein, 44 aa, Artificial Sequence
  Synthetic Polypeptide
  DISULFID (1)..(5)
  DISULFID (14)..(32)
  MOD_RES (16)..(16): Xaa = homoglutamic acid
CDATCQFRKAIDDCQXQAHHSNVPGNSVFKECMKQKKKEFKAGK

SEQ ID NO: 352 - protein, 44 aa, Artificial Sequence
  Synthetic Polypeptide
  DISULFID (1)..(5)
  DISULFID (14)..(32)
CDATCQFRKAIDDCQRQAHHSNVPGNSVFKECMKQKKKEFKAGK

SEQ ID NO: 353 - protein, 44 aa, Artificial Sequence
  Synthetic Polypeptide
  DISULFID (1)..(5)
  DISULFID (14)..(32)
  MOD_RES (15)..(15): Xaa = citrulline
CDATCQFRKAIDDCXKQAHHSNVPGNSVFKECMKQKKKEFKAGK

SEQ ID NO: 354 - protein, 44 aa, Artificial Sequence
  Synthetic Polypeptide
  DISULFID (1)..(5)
  DISULFID (14)..(32)
CDATCQFRKAIDDCDKQAHHSNVPGNSVFKECMKQKKKEFKAGK

SEQ ID NO: 355 - protein, 44 aa, Artificial Sequence
  Synthetic Polypeptide
  DISULFID (1)..(5)
  DISULFID (14)..(32)
CDATCQFRKAIDDCQKQAHYSNVPGNSVFKECMKQKKKEFKAGK

SEQ ID NO: 356 - protein, 44 aa, Artificial Sequence
  Synthetic Polypeptide
  DISULFID (1)..(5)
  DISULFID (14)..(32)
CDATCQFRKAIDDCQKQAYHSNVPGNSVFKECMKQKKKEFKAGK

SEQ ID NO: 357 - protein, 44 aa, Artificial Sequence
  Synthetic Polypeptide
  DISULFID (1)..(5)
  DISULFID (14)..(32)
CDATCQFRKAIDDCQKQAHHVNVPGNSVFKECMKQKKKEFKAGK

SEQ ID NO: 358 - protein, 44 aa, Artificial Sequence
  Synthetic Polypeptide
  DISULFID (1)..(5)
  DISULFID (14)..(32)
CDATCQFRKAIDDCQKQAHHSNTPGNSVFKECMKQKKKEFKAGK

SEQ ID NO: 359 - protein, 44 aa, Artificial Sequence
  Synthetic Polypeptide
  DISULFID (1)..(5)
  DISULFID (14)..(32)
CDATCQFRKAIDDCQKQAHHSNVPGNSTFKECMKQKKKEFKAGK

SEQ ID NO: 360 - protein, 44 aa, Artificial Sequence
  Synthetic Polypeptide
  DISULFID (1)..(5)
  DISULFID (14)..(32)
CDATCQFRKAIDDCQKQLHHSNVPGNSVFKECMKQKKKEFKAGK

SEQ ID NO: 361 - protein, 44 aa, Artificial Sequence
  Synthetic Polypeptide
  DISULFID (1)..(5)
  DISULFID (14)..(32)
CDATCQFRKLIDDCQKQAHHSNVPGNSVFKECMKQKKKEFKAGK

SEQ ID NO: 362 - protein, 43 aa, Artificial Sequence
  Synthetic Polypeptide
  DISULFID (1)..(5)
  DISULFID (14)..(31)
CDATCQFRKAIDDCQKQAHHSNVPGNSVKECMKQKKKEFKAGK

SEQ ID NO: 363 - protein, 43 aa, Artificial Sequence
  Synthetic Polypeptide
  DISULFID (1)..(5)
  DISULFID (14)..(31)
CDATCQFRKAIDDCQKQAHHSNVPGNSFKECMKQKKKEFKAGK

SEQ ID NO: 364 - protein, 43 aa, Artificial Sequence
  Synthetic Polypeptide
  DISULFID (1)..(5)
  DISULFID (14)..(31)
CDATCQFRKAIDDCQKQAHHSNVPGSVFKECMKQKKKEFKAGK

SEQ ID NO: 365 - protein, 43 aa, Artificial Sequence
  Synthetic Polypeptide
  DISULFID (1)..(5)
  DISULFID (14)..(31)
CDATCQFRKAIDDCQKQAHHSNVPNSVFKECMKQKKKEFKAGK

SEQ ID NO: 366 - protein, 44 aa, Artificial Sequence; identical to SEQ ID NO: 334
  Synthetic Polypeptide
  DISULFID (1)..(5)
  DISULFID (14)..(32)
  MOD_RES (24)..(24): Xaa = sarcosine

SEQ ID NO: 367 - protein, 44 aa, Artificial Sequence; identical to SEQ ID NO: 334
  Synthetic Polypeptide
  DISULFID (1)..(5)
  DISULFID (14)..(32)
  MOD_RES (24)..(24): Xaa = 4-hydroxyproline

SEQ ID NO: 368 - protein, 44 aa, Artificial Sequence
  Synthetic Polypeptide
  DISULFID (1)..(5)
  DISULFID (14)..(32)
CDATCQFRKAIDECQKQAHHSNVPGNSVFKECMKQKKKEFKAGK

SEQ ID NO: 369 - protein, 44 aa, Artificial Sequence
  Synthetic Polypeptide
  DISULFID (1)..(5)
  DISULFID (14)..(32)
CDATCQFRKAIEDCQKQAHHSNVPGNSVFKECMKQKKKEFKAGK

SEQ ID NO: 370 - protein, 44 aa, Artificial Sequence
  Synthetic Polypeptide
  DISULFID (1)..(5)
  MOD_RES (6)..(6): Xaa = citrulline
  DISULFID (14)..(32)
CDATCXFRKAIDDCQKQAHHSNVPGNSVFKECMKQKKKEFKAGK

SEQ ID NO: 371 - protein, 44 aa, Artificial Sequence
  Synthetic Polypeptide
  DISULFID (1)..(5)
  DISULFID (14)..(32)
CDATCKFRKAIDDCQKQAHHSNVPGNSVFKECMKQKKKEFKAGK

SEQ ID NO: 372 - protein, 44 aa, Artificial Sequence
  Synthetic Polypeptide
  DISULFID (1)..(5)
  DISULFID (14)..(32)
CDATCEFRKAIDDCQKQAHHSNVPGNSVFKECMKQKKKEFKAGK

SEQ ID NO: 373 - protein, 44 aa, Artificial Sequence
  Synthetic Polypeptide
  DISULFID (1)..(5)
  DISULFID (14)..(32)
CDATCNFRKAIDDCQKQAHHSNVPGNSVFKECMKQKKKEFKAGK

SEQ ID NO: 374 - protein, 44 aa, Artificial Sequence
  Synthetic Polypeptide
  DISULFID (1)..(5)
  DISULFID (14)..(32)
CDATCQYRKAIDDCQKQAHHSNVPGNSVFKECMKQKKKEFKAGK

SEQ ID NO: 375 - protein, 44 aa, Artificial Sequence
  Synthetic Polypeptide
  DISULFID (1)..(5)
  DISULFID (14)..(32)
CDATCQFKRAIDDCQKQAHHSNVPGNSVFKECMKQKKKEFKAGK

SEQ ID NO: 376 - protein, 44 aa, Artificial Sequence
  Synthetic Polypeptide
  DISULFID (1)..(5)
  DISULFID (14)..(32)
CDASCQFRKAIDDCQKQAHHSNVPGNSVFKECMKQKKKEFKAGK

SEQ ID NO: 377 - protein, 44 aa, Artificial Sequence
  Synthetic Polypeptide
  DISULFID (1)..(5)
  DISULFID (14)..(32)
CDAVCQFRKAIDDCQKQAHHSNVPGNSVFKECMKQKKKEFKAGK

SEQ ID NO: 378 - protein, 44 aa, Artificial Sequence
  Synthetic Polypeptide
  DISULFID (1)..(5)
  MOD_RES (3)..(3): Xaa = 2-aminoisobutyric acid
  DISULFID (14)..(32)
CDXTCQFRKAIDDCQKQAHHSNVPGNSVFKECMKQKKKEFKAGK

SEQ ID NO: 379 - protein, 44 aa, Artificial Sequence
  Synthetic Polypeptide
  DISULFID (1)..(5)
  DISULFID (14)..(32)
CDPTCQFRKAIDDCQKQAHHSNVPGNSVFKECMKQKKKEFKAGK

SEQ ID NO: 380 - protein, 44 aa, Artificial Sequence
  Synthetic Polypeptide
  DISULFID (1)..(5)
  DISULFID (14)..(32)
CEATCQFRKAIDDCQKQAHHSNVPGNSVFKECMKQKKKEFKAGK

SEQ ID NO: 381 - protein, 44 aa, Artificial Sequence
  Synthetic Polypeptide
  DISULFID (14)..(32)
SDATSQFRKAIDDCQKQAHHSNVPGNSVFKECMKQKKKEFKAGK

SEQ ID NO: 382 - protein, 44 aa, Artificial Sequence
  Synthetic Polypeptide
  DISULFID (1)..(5)
  DISULFID (14)..(32)
  MOD_RES (34)..(34): Xaa = 2-aminoisobutyric acid
CDATCQFRKAIDDCQKQAHHSNVPGNSVFKECMXQKKKEFKAGK

SEQ ID NO: 383 - protein, 44 aa, Artificial Sequence
  Synthetic Polypeptide
  DISULFID (1)..(5)
  DISULFID (14)..(32)
  MOD_RES (31)..(31): Xaa = 2-aminoisobutyric acid
CDATCQFRKAIDDCQKQAHHSNVPGNSVFKXCMKQKKKEFKAGK

SEQ ID NO: 384 - protein, 44 aa, Artificial Sequence
  Synthetic Polypeptide
  DISULFID (1)..(5)
  DISULFID (14)..(32)
  MOD_RES (30)..(30): Xaa = 2-aminoisobutyric acid
CDATCQFRKAIDDCQKQAHHSNVPGNSVFXECMKQKKKEFKAGK

SEQ ID NO: 385 - protein, 44 aa, Artificial Sequence
  Synthetic Polypeptide
  DISULFID (1)..(5)
  DISULFID (14)..(32)
  MOD_RES (29)..(29): Xaa = 2-aminoisobutyric acid
CDATCQFRKAIDDCQKQAHHSNVPGNSVXKECMKQKKKEFKAGK

SEQ ID NO: 386 - protein, 44 aa, Artificial Sequence
  Synthetic Polypeptide
  DISULFID (1)..(5)
  DISULFID (14)..(32)
  MOD_RES (21)..(21): Xaa = 2-aminoisobutyric acid
CDATCQFRKAIDDCQKQAHHXNVPGNSVFKECMKQKKKEFKAGK

SEQ ID NO: 387 - protein, 44 aa, Artificial Sequence
  Synthetic Polypeptide
  DISULFID (1)..(5)
  DISULFID (14)..(32)
CDATCQFRKAIDDCQKQAHHSNVPGNSVFAECMKQKKKEFKAGK

SEQ ID NO: 388 - protein, 44 aa, Artificial Sequence
  Synthetic Polypeptide
  DISULFID (1)..(5)
  DISULFID (14)..(32)
CDATCQFRKAIDDCQKQAHHSNVPGNSVFKACMKQKKKEFKAGK

SEQ ID NO: 389 - protein, 44 aa, Artificial Sequence
  Synthetic Polypeptide
  DISULFID (1)..(5)
  DISULFID (14)..(32)
CDATCQFRKAIDDCQKQAHHSNVPGNSVFKECMKQKKKEFKAEK

SEQ ID NO: 390 - protein, 44 aa, Artificial Sequence
  Synthetic Polypeptide
  DISULFID (1)..(5)
  DISULFID (14)..(32)
CDATCQFRKAIDDCQKQAHHSNVPGNSVFKECMKQKKKEFKEGK

SEQ ID NO: 391 - protein, 44 aa, Artificial Sequence
  Synthetic Polypeptide
  DISULFID (1)..(5)
  DISULFID (14)..(32)
CDATCQFRKAIDDCQKQAHHSNVPGNSVFKECMKQKKKAFKAGK

SEQ ID NO: 392 - protein, 44 aa, Artificial Sequence
  Synthetic Polypeptide
  DISULFID (1)..(5)
  DISULFID (14)..(32)
CDATCQFRKAIDDCQKQAHHSNVPGNSVFKECMKQKAKEFKAGK

SEQ ID NO: 393 - protein, 44 aa, Artificial Sequence
  Synthetic Polypeptide
  DISULFID (1)..(5)
  DISULFID (14)..(32)
CDATCQFRKAIDDCQKQAHHSNVPGNSVFKECMKAKKKEFKAGK

SEQ ID NO: 394 - protein, 44 aa, Artificial Sequence
  Synthetic Polypeptide
  DISULFID (1)..(5)
  DISULFID (14)..(32)
CDATCQFRKAIDDCQKQAHHSNVPGNSVFKECMAQKKKEFKAGK

SEQ ID NO: 395 - protein, 44 aa, Artificial Sequence
  Synthetic Polypeptide
  DISULFID (1)..(5)
  DISULFID (14)..(32)
CDATCQFRKAIDDCQKQAHHSNVPGNSVFKECAKQKKKEFKAGK

SEQ ID NO: 396 - protein, 40 aa, Artificial Sequence
  Synthetic Polypeptide
  DISULFID (1)..(5)
  DISULFID (14)..(28)
CDATCQFRKAIDDCQKQAHHSNSVFKECMKQKKKEFKAGK

SEQ ID NO: 397 - protein, 41 aa, Artificial Sequence
  Synthetic Polypeptide
  DISULFID (1)..(5)
  DISULFID (14)..(29)
CDATCQFRKAIDDCQKQAHHSNVSVFKECMKQKKKEFKAGK

SEQ ID NO: 398 - protein, 43 aa, Artificial Sequence
  Synthetic Polypeptide
  DISULFID (1)..(5)
  DISULFID (14)..(31)
CDATCQFRKAIDDCQKQAHHSNVGNSVFKECMKQKKKEFKAGK

SEQ ID NO: 399 - protein, 44 aa, Artificial Sequence
  Synthetic Polypeptide
  DISULFID (1)..(5)
  DISULFID (14)..(32)
  MOD_RES (33)..(33): Xaa = norleucine
CDATCQFRKAIDDCQKQAHHSNVPGNSVFKECXKQKKKEFKAGK

SEQ ID NO: 400 - protein, 44 aa, Artificial Sequence
  Synthetic Polypeptide
  DISULFID (1)..(5)
  DISULFID (14)..(32)
  MOD_RES (43)..(43): Xaa = 2-aminoisobutyric acid
CDATCQFRKAIDDCQKQAHHSNVPGNSVFKECMKQKKKEFKAXK

SEQ ID NO: 401 - protein, 44 aa, Artificial Sequence
  Synthetic Polypeptide
  DISULFID (1)..(5)
  DISULFID (14)..(32)
  MOD_RES (42)..(42): Xaa = 2-aminoisobutyric acid
CDATCQFRKAIDDCQKQAHHSNVPGNSVFKECMKQKKKEFKXGK

SEQ ID NO: 402 - protein, 44 aa, Artificial Sequence; identical to SEQ ID NO: 318
  Synthetic Polypeptide
  DISULFID (1)..(5)
  DISULFID (14)..(32)
  MOD_RES (41)..(41): Xaa = 2-aminoisobutyric acid

SEQ ID NO: 403 - protein, 44 aa, Artificial Sequence; identical to SEQ ID NO: 312
  Synthetic Polypeptide
  DISULFID (1)..(5)
  DISULFID (14)..(32)
  MOD_RES (40)..(40): Xaa = 2-aminoisobutyric acid

SEQ ID NO: 404 - protein, 44 aa, Artificial Sequence
  Synthetic Polypeptide
  DISULFID (1)..(5)
  DISULFID (14)..(32)
  MOD_RES (39)..(39): Xaa = 2-aminoisobutyric acid
CDATCQFRKAIDDCQKQAHHSNVPGNSVFKECMKQKKKXFKAGK

SEQ ID NO: 405 - protein, 44 aa, Artificial Sequence
  Synthetic Polypeptide
  DISULFID (1)..(5)
  DISULFID (14)..(32)
  MOD_RES (38)..(38): Xaa = 2-aminoisobutyric acid
CDATCQFRKAIDDCQKQAHHSNVPGNSVFKECMKQKKXEFKAGK

SEQ ID NO: 406 - protein, 44 aa, Artificial Sequence
  Synthetic Polypeptide
  DISULFID (1)..(5)
  DISULFID (14)..(32)
  MOD_RES (37)..(37): Xaa = 2-aminoisobutyric acid
CDATCQFRKAIDDCQKQAHHSNVPGNSVFKECMKQKXKEFKAGK

SEQ ID NO: 407 - protein, 44 aa, Artificial Sequence; identical to SEQ ID NO: 322
  Synthetic Polypeptide
  DISULFID (1)..(5)
  DISULFID (14)..(32)
  MOD_RES (36)..(36): Xaa = 2-aminoisobutyric acid

SEQ ID NO: 408 - protein, 44 aa, Artificial Sequence
  Synthetic Polypeptide
  DISULFID (1)..(5)
  DISULFID (14)..(32)
  MOD_RES (20)..(20): Xaa = 2-aminoisobutyric acid
CDATCQFRKAIDDCQKQAHXSNVPGNSVFKECMKQKKKEFKAGK

SEQ ID NO: 409 - protein, 44 aa, Artificial Sequence
  Synthetic Polypeptide
  DISULFID (1)..(5)
  DISULFID (14)..(32)
  MOD_RES (19)..(19): Xaa = 2-aminoisobutyric acid
CDATCQFRKAIDDCQKQAXHSNVPGNSVFKECMKQKKKEFKAGK

SEQ ID NO: 410 - protein, 44 aa, Artificial Sequence
  Synthetic Polypeptide
  DISULFID (1)..(5)
  DISULFID (14)..(32)
  MOD_RES (18)..(18): Xaa = 2-aminoisobutyric acid
CDATCQFRKAIDDCQKQXHHSNVPGNSVFKECMKQKKKEFKAGK

SEQ ID NO: 411 - protein, 44 aa, Artificial Sequence; identical to SEQ ID NO: 348
  Synthetic Polypeptide
  DISULFID (1)..(5)
  DISULFID (14)..(32)
  MOD_RES (17)..(17): Xaa = 2-aminoisobutyric acid

SEQ ID NO: 412 - protein, 44 aa, Artificial Sequence; identical to SEQ ID NO: 351
  Synthetic Polypeptide
  DISULFID (1)..(5)
  DISULFID (14)..(32)
  MOD_RES (16)..(16): Xaa = 2-aminoisobutyric acid

SEQ ID NO: 413 - protein, 36 aa, Artificial Sequence
  Synthetic Polypeptide
  DISULFID (1)..(5)
  DISULFID (14)..(32)
  MOD_RES (36)..(36): C-terminal amidation
CDATCQFRKAIDDCQKQAHHSNVPGNSVFKECMKQK

SEQ ID NO: 414 - protein, 37 aa, Artificial Sequence
  Synthetic Polypeptide
  DISULFID (1)..(5)
  DISULFID (14)..(32)
  MOD_RES (37)..(37): C-terminal amidation
CDATCQFRKAIDDCQKQAHHSNVPGNSVFKECMKQKK

SEQ ID NO: 415 - protein, 38 aa, Artificial Sequence
  Synthetic Polypeptide
  DISULFID (1)..(5)
  DISULFID (14)..(32)
  MOD_RES (38)..(38): C-terminal amidation
CDATCQFRKAIDDCQKQAHHSNVPGNSVFKECMKQKKK

SEQ ID NO: 416 - protein, 39 aa, Artificial Sequence
  Synthetic Polypeptide
  DISULFID (1)..(5)
  DISULFID (14)..(32)
  MOD_RES (39)..(39): C-terminal amidation
CDATCQFRKAIDDCQKQAHHSNVPGNSVFKECMKQKKKE

SEQ ID NO: 417 - protein, 40 aa, Artificial Sequence
  Synthetic Polypeptide
  DISULFID (1)..(5)
  DISULFID (14)..(32)
  MOD_RES (40)..(40): C-terminal amidation
CDATCQFRKAIDDCQKQAHHSNVPGNSVFKECMKQKKKEF

SEQ ID NO: 418 - protein, 41 aa, Artificial Sequence; identical to SEQ ID NO: 313
  Synthetic Polypeptide
  DISULFID (1)..(5)
  DISULFID (14)..(32)
  MOD_RES (41)..(41): C-terminal amidation

SEQ ID NO: 419 - skipped

SEQ ID NO: 420 - protein, 43 aa, Artificial Sequence; identical to SEQ ID NO: 273
  Synthetic Polypeptide
  DISULFID (1)..(5)
  DISULFID (14)..(32)
  MOD_RES (43)..(43): C-terminal amidation

SEQ ID NO: 421 - protein, 44 aa, Artificial Sequence
  Synthetic Polypeptide
  DISULFID (1)..(5)
  DISULFID (14)..(32)
CDATCQFRKAIDDCQKQAHHSNVPGNSVFKECMKQKKKEFKAGA

SEQ ID NO: 422 - protein, 44 aa, Artificial Sequence
  Synthetic Polypeptide
  DISULFID (1)..(5)
  DISULFID (14)..(32)
CDATCQFRKAIDDCQKQAHHSNVPGNSVFKECMKQKKKEFKAGE

SEQ ID NO: 423 - skipped

SEQ ID NO: 424 - protein, 43 aa, Artificial Sequence
  Synthetic Polypeptide
  DISULFID (1)..(5)
  DISULFID (14)..(31)
  MOD_RES (43)..(43): C-terminal amidation
CDATCQFRKAIDDCAHRAWHSNVPGSVFKLCMKQKKKEWKAGH

SEQ ID NO: 425 - protein, 43 aa, Artificial Sequence
  Synthetic Polypeptide
  DISULFID (1)..(5)
  DISULFID (14)..(31)
  MOD_RES (43)..(43): C-terminal amidation
CDATCQFRKAIDDCAGRASHANVPGSVFKACMKQKKKEWKAGH

SEQ ID NO: 426 - protein, 42 aa, Artificial Sequence
  Synthetic Polypeptide
  DISULFID (14)..(31)
  MOD_RES (42)..(42): C-terminal amidation
SDATSQYRKGLVACLYKKVAMQKRYSVFKACMKQKKKEWKAG

SEQ ID NO: 427 - protein, 39 aa, Artificial Sequence
  Synthetic Polypeptide
  DISULFID (1)..(5)
  DISULFID (14)..(31)
  MOD_RES (39)..(39): C-terminal amidation
CDATCQYRKGLVACLYKKVAMQKRYSVFKACMKQKKKEW

SEQ ID NO: 428 - protein, 38 aa, Artificial Sequence
  Synthetic Polypeptide
  DISULFID (1)..(5)
  DISULFID (14)..(27)
  PEPTIDE (38)..(38): C-term amide
CDATCQFRKAIDDCARQAYHASVFKACMKQKKKEWKAG

SEQ ID NO: 429 - protein, 39 aa, Artificial Sequence
  Synthetic Polypeptide
  DISULFID (1)..(5)
  DISULFID (14)..(28)
  PEPTIDE (39)..(39): C-term amide
CDATCQFRKAIDDCARQAYHSNSVFKACMKQKKKEWKAG

SEQ ID NO: 430 - protein, 38 aa, Artificial Sequence
  Synthetic Polypeptide
  DISULFID (1)..(5)
  DISULFID (14)..(27)
  PEPTIDE (38)..(38): C-term amide
CDATCQFRKAIDDCARQAYHSSVFKSCMKQKKKEWKAG

SEQ ID NO: 431 - protein, 38 aa, Artificial Sequence
  Synthetic Polypeptide
  DISULFID (1)..(5)
  DISULFID (14)..(27)
  PEPTIDE (38)..(38): C-term amide
CDATCQFRKAIDDCARSAYHSSVFKACMKQKKKEWKAG

SEQ ID NO: 432 - protein, 38 aa, Artificial Sequence
  Synthetic Polypeptide
  DISULFID (1)..(5)
  DISULFID (14)..(27)
  PEPTIDE (38)..(38): C-term amide
CDATCQFRKAIDDCARQSYHSSVFKACMKQKKKEWKAG

SEQ ID NO: 433 - protein, 38 aa, Artificial Sequence
  Synthetic Polypeptide
  DISULFID (1)..(5)
  DISULFID (14)..(27)
  PEPTIDE (38)..(38): C-term amide
CDATCQFRKAIDDCARQASHSSVFKACMKQKKKEWKAG

SEQ ID NO: 434 - protein, 38 aa, Artificial Sequence
  Synthetic Polypeptide
  DISULFID (1)..(5)
  DISULFID (14)..(27)
  PEPTIDE (38)..(38): C-term amide
CDATCQFRKAIDDCARQAKHSSVFKACMKQKKKEWKAG

SEQ ID NO: 435 - protein, 38 aa, Artificial Sequence
  Synthetic Polypeptide
  DISULFID (1)..(5)
  DISULFID (14)..(27)
  PEPTIDE (38)..(38): C-term amide
CDATCQFRKAIDDCARQAYHSSVFKACLKQKKKEWKAG

SEQ ID NO: 436 - protein, 38 aa, Artificial Sequence
  Synthetic Polypeptide
  DISULFID (1)..(5)
  DISULFID (14)..(27)
  PEPTIDE (38)..(38): C-term amide
CDATCQFRKAIDDCARQAYHSSVFKSCLKQKKKEWKAG

SEQ ID NO: 437 - protein, 25 aa, Artificial Sequence
  Synthetic Polypeptide
  DISULFID (1)..(5)
  PEPTIDE (25)..(25): C-term amide
CDATCQYRKGLVASLYKKVAMQKRY

SEQ ID NO: 438 - protein, 30 aa, Artificial Sequence
  Synthetic Polypeptide
  DISULFID (1)..(5)
CDATCQYRKGLVASVFKASMKQKKKEFKAG

SEQ ID NO: 439 - protein, 37 aa, Artificial Sequence
  Synthetic Polypeptide
  DISULFID (1)..(5)
  DISULFID (14)..(25)
CDATCQFRKAIDDCARQAYHSFKACMKQKKKEWKAGH

SEQ ID NO: 440 - protein, 34 aa, Artificial Sequence
  Synthetic Polypeptide
  DISULFID (12)..(25)
ATSQFRKAIDDCARQAYHSSVFKACMKQKKKEWK

SEQ ID NO: 441 - protein, 32 aa, Artificial Sequence
  Synthetic Polypeptide
  DISULFID (10)..(21)
SDATSQFRKCIDDSGAFKASCKQKKKEWKAGH

SEQ ID NO: 442 - protein, 31 aa, Artificial Sequence
  Synthetic Polypeptide
  DISULFID (1)..(30)
CDATSQFRKAIDDSAFKASMKQKKKEWKACH

SEQ ID NO: 443 - protein, 32 aa, Artificial Sequence
  Synthetic Polypeptide
  DISULFID (1)..(5)
  DISULFID (14)..(20)
CDATCQFRKAIDDCAAFKACMKQKKKEWKAGH

SEQ ID NO: 444 - protein, 31 aa, Artificial Sequence
  Synthetic Polypeptide
  DISULFID (1)..(5)
  DISULFID (14)..(19)
CDATCQFRKAIDDCAFKACMKQKKKEWKAGH

SEQ ID NO: 445 - protein, 43 aa, Artificial Sequence
  Synthetic Polypeptide
  DISULFID (1)..(5)
  DISULFID (14)..(31)
  PEPTIDE (43)..(43): C-term amide
CDATCQFRKAIDDCANKSWHSNVPGSVFKLCMKQKKKEWKAGH

SEQ ID NO: 446 - protein, 42 aa, Artificial Sequence
  Synthetic Polypeptide
  DISULFID (1)..(5)
  DISULFID (14)..(31)
  PEPTIDE (42)..(42): C-term amide
CDATCQFRKAIDDCAGTARHSNVPGSVFKACMKQKKKEWKAG

SEQ ID NO: 447 - protein, 33 aa, Artificial Sequence
  Synthetic Polypeptide
  DISULFID (1)..(5)
  DISULFID (14)..(21)
CDATCQFRKAIDDCARQFKACMKQKKKEWKAGH

SEQ ID NO: 448 - protein, 35 aa, Artificial Sequence
  Synthetic Polypeptide
  DISULFID (1)..(5)
  DISULFID (14)..(23)
CDATCQFRKAIDDCARQAYFKACMKQKKKEWKAGH

SEQ ID NO: 449 - protein, 35 aa, Artificial Sequence
  Synthetic Polypeptide
  DISULFID (1)..(5)
  DISULFID (14)..(23)
CDATCQFRKAIDDCARQAYHSACMKQKKKEWKAGH

SEQ ID NO: 450 - protein, 35 aa, Artificial Sequence
  Synthetic Polypeptide
  DISULFID (1)..(5)
  DISULFID (14)..(25)
CDATCQFRKAIDDCARQAYHSFKACMKQKKKEWKH

SEQ ID NO: 451 - protein, 36 aa, Artificial Sequence
  Synthetic Polypeptide
  DISULFID (1)..(5)
  DISULFID (14)..(25)
CDATCQFRKAIDDCARQAYHSFKACMKQKKKEWKAH